European Patent Application EP 4 253 567 A1, published October 4, 2023. Title: A method of predicting risk of an aggressive or recurrent cancer. Applicant: OncoAssure Limited. The sequence listing filed with the application follows.

SEQUENCE LISTING (16 sequences)

SEQ ID NO: 1 - DNA, 8182 bp, Homo sapiens
aggcgggaattcgtctcgggttgtgtggttgaggggtctggtgggtcgaggaaaggtaacggcggccccagtcctgcacacaaggccggggaagtagcagcacccccaggaagagggaggaggaagggctcgtgccctttcttctcttccagggctccgctttatttgctctcagaagtcggtttcctttccttttcttcagtgaatcggagctcagagcgttgcttcggtttccctccagacagttaggaatctgaaataaacaggaaagcactatgtcttcaatgtggtctgaatatacaattggtggggtgaagatttactttccttataaagcttacccgtcacagcttgctatgatgaattctattctcagaggattaaacagcaagcaacattgtttgttggagagtcccacaggaagtggaaaaagcttagccttactttgttctgctttagcatggcaacaatctcttagtgggaaaccagcagatgagggcgtaagtgaaaaagctgaagtacaattgtcatgttgttgtgcatgccattcaaaggattttacaaacaatgacatgaaccaaggaacttcacgtcatttcaactatccaagcacaccaccttctgaaagaaatggcacttcatcaacttgtcaagactcccctgaaaaaaccactctggctgcaaagttatctgctaagaaacaggcatccatatacagagatgaaaatgatgattttcaagtagagaagaaaagaattcgacccttagaaactacacagcagattagaaaacgtcattgctttggaacagaagtacacaatttggatgcaaaagttgattcaggaaagactgtaaaactcaactctccactggaaaagataaactccttttcgccacagaaaccccctggccactgttctaggtgctgttgttctactaaacaaggaaacagtcaagagtcatcgaataccattaagaaggatcatacagggaaatccaagatacccaaaatatattttgggacacgcacacacaagcagattgctcagattactagagagctccggaggacggcatattcaggggttccaatgactattctttccagcagggatcatacttgtgtccatcctgaggtagtcggtaacttcaacagaaatgagaagtgcatggaattgctagatgggaaaaacggaaaatcctgctatttttatcatggagttcataaaattagtgatcagcacacattacagactttccaagggatgtgcaaagcctgggatatagaagaacttgtcagcctggggaagaaactaaaggcctgtccatattacacagcccgagaactaatacaagatgctgacatcatattttgtccctacaactatcttctagatgcacaaataagggaaagtatggatttaaatctgaaagaacaggttgtcattttagatgaagctcataacatcgaggactgtgctcgggaatcagcaagttacagtgtaacagaagttcagcttcggtttgctcgggatgaactagatagtatggtcaacaataatataaggaagaaagatcatgaacccctacgagctgtgtgctgtagcctcattaattggttagaagcaaacgctgaatatcttgtagaaagagattatgaatcagcttgtaaaatatggagtggaaatgaaatgctcttaactttacacaaaatgggtatcaccactgctacttttcccattttgcagggacatttttctgctgttcttcaaaaagaggaaaaaatctcaccaatttatggtaaagaggaggcaagagaagtacctgttattagtgcatcaactcaaataatgcttaaaggactttttatggtacttgactatctttttaggcaaaatagcagatttgcagatgattataaaattgcgattcaacagacttactcctggacaaatcagattgatatttcagacaaaaatgggttgttggttctaccaaaaaataagaaacgttcacgacagaaaactgcagttcatgtgctaaacttttggtgcttaaatccagctgtggccttttcagatattaatggcaaagttcagaccattgttttgacatctggtacattatcaccaatgaaatccttttcgtcagaacttggtgttacatttactatccagctggaggctaatcatatcattaaaaattcacaggtttgggttggtaccattgggtcaggccccaagggtcggaatctctgtgctaccttccagaatactgaaacatttgagttccaagatgaagtgggagcacttttgttatctgtgtgccagactgtgagccaaggaattttgtgtttcttgccatcttacaagttattagaaaaattaaaagaacgttggctctctactggtttatggcataatctggagttggtgaagacagtcattgtagaaccacagggaggagaaaaaacaaattttgatgaattactgcaggtgtactatgacgcaatcaaatacaaaggagagaaagatggagctctcctggtagcagtttgtcgtggtaaagtgagtgagggtctggatttctcagatgacaatgcccgtgctgtcataacaataggaattccttttccaaatgtgaaagatctacaggttgaactaaaacgacaatacaatgaccaccattcaaaattgagaggtcttctacctggccgtcagtggtatgaaattcaagcatacagggccttaaaccaggcccttggtagatgtattagacacagaaatgattggggagctcttattctagtggatgatcgctttaggaataacccaagtcgctatatatctggactttctaaatgggtacggcagcagattcagcaccattcaacctttgaaagtgcactggaatccttggctgaattttccaaaaagcatcaaaaagttcttaatgtatccataaaggacagaaccaatatacaggacaatgagtctacacttgaagtgacctctttaaagtacagtacctcaccttatttactggaagcagcaagtcatctatcaccagaaaattttgtggaagatgaagcaaagatatgtgtccaggaactacagtgtcctaaaattattaccaaaaattcacctctaccaagtagcattatctccagaaaggagaaaaatgatccagtattcctggaagaagcagggaaagcagaaaaaattgtgatttccagatccacaagcccaactttcaacaaacaaacaaagagagttagctggtcaagctttaattctttgggacagtattttactggtaaaataccgaaggcaacacctgagctcgggtcatcagagaatagtgcctctagtcctccccgtttcaaaacagagaagatggaaagtaaaactgttttgcccttcactgataaatgtgaatcctcaaatctgacagtaaacacatcgtttggatcatgccctcaatcagaaaccattatttcatcattaaagattgatgccacccttactagaaaaaatcattctgaacatccgctctgttctgaagaagccctggatccagacattgaattgtctctagtaagtgaagaagataaacagtccacttcaaatagagattttgaaacagaagcagaagatgaatctatctattttacacctgaactttatgatcctgaagatacagatgaagaaaaaaatgacctagctgaaactgatagaggaaatagattggctaacaattcagattgcattttagctaaagacctttttgaaattagaactataaaagaagtagattcagccagagaagtgaaagctgaggattgcatagatacaaagttgaatggaattctgcatattgaagaaagtaaaattgatgacattgatggtaatgtaaaaacaacttggataaatgaactggaactgggaaaaactcatgaaatagaaataaagaactttaaaccatctccttccaaaaataaaggcatgtttcctggttttaagtaataatacttaactctcaagctaagtaaaaatatgtcatcatgcttatgttaaactctgttgtaagtaataatttgtaaattgaataagtggcatactttttaaaaaactattttatgttcagaaatgtaaatgttattattcttgagtttttgggtttttttttttgagacagagtcttggtctgttgcccaggctggaatgcagtggtgtgctctgggctcactgcaaccttcacctccaggttcaagtgattctcctgcctcagccttctgagtagctgggactacaggtgtgcaccaccatgcccagctagtttttgtatttttagtagagatggggtttcaccatgttggccaggctggtctcgaactcctggcctcgtgatctgcccttctctgcctccctaagttgctgggattacaggtgtgagccacagtgcctggcccattcttgagttttgataaagtaattcatacaaagtactgtcctcaaataagtcttccttagctaaatgcaatttaaaattattcaaagatcctagggcacttctagtttcacgtaaatattcatattaggtggttctcttcatccatttgttttcacactgatacataaaaattaacagcagtctaatctagtgacacctcagtcatatttcgctatagattttacctcaaatcagtccaagactttttcagagatcaccatttgtcttgaaaggtttatttcgttattaaactgcctacttataagtaattaagagaaattaagaaagtagtatgcatttttaattgaaattgttttacattctttgtataataaacctaaaaccaaacatgtcataaacaaattgacgtaaagatataaaatgccaaatgaagtattccaaattttctattctaattatttagcttcaccatcattgtggaaaaaaatactagatcctgcttagtattatatatttttcctagtggatcagtgagtaataagtaccaaacactagactagaaggtaatttctacattgtttagaaagggtgaaacaatttatcccctctggtattgttctagcataagctttagttatacaatgattaagatagaaaacttcatatataaatttgataagcaaacccacatttatagctgcagctaaaatatgtttccttagggcacagtaatcctttctgtgaattttgaccttgtttgtgtttttgtgaatgaagctatatgtctaatcaaaaatgattataaaagaggctcatctctgacatcattccaaaaatacattcattgatctctttttaagaaacatctgttattcactgggcattgggactttttgtgagtaatttgaattgaaattttatgagctatccaagaattctgtatggtctattattttcaagtcaaaatttccagtaaggatttactttacatttcatttggataaatgaatcattatataggtatgtctttgcttccattttgagacatttagatttttacagcctgtttctatagcatttgatgttacaactctaagcgtagttcaaagacatttaaattgacaagttaccagttaaagaatttagaatatattagatcccatctagtattatatattttttctagttgatcattgagcagtaaataccaaatactcgattagaaggtaatttttacattgttttgaaagggtgaaacaatttatctcctctggtattattcttaaaccacagatagggatagtagggtagtgaaacgaataaatacctggtagaagacaagagacttgggctctacacctggctctgccactgatttgctaagtcatattggcaatcaccacacccttcagggaattagtttcatctgtaaaatgcagcggttagtactataaaatcatacaaatttctttgtgctttgagaatctataaaggaatgtctgttgatattctgagtcgattttcatttgcttttgttccagaacggttaaaataaagcatattatttcatttaaaaagtaaagtggctcttactcatttacatttagggaacgatggtgacgtggtttggctatgtccccagccagatctcatcttgaattgtagttcccataatcccgacgtgttgtgggaaggacccagtgggaggtaattgaatcgtgggggcggttaccctcatgcggttctcgtgatactgagttcttatgagacctgatgattttataaggagcttttccctgcttcactctcattcttctctcctgctgccctgtgaaaagttgccttccgccatgattgtaagtttcttgaggcctcctcagtcatgcagaactgtgagtcaattaaacctctttcctttataaattacccagtcttgggtatgactttattagcagcatgagaacagactgacacagatggtatatgtgcataataacttggaaagctagatatttattttcgcaatgctacaattaaaacattttgaggacttttaaaattacctttagggccaggcgcggtggctcacgcctgtaatcccagcactttgggaggccgaggcgggcggatcacgaggtcaggagatcgagaccatcctggttaacacggtgaaaccccgtctctactaaaaatacaaaaaattagccaggcgtggtggcgggcgcctgtagtcccagctactcaggaggctgaggcaggagaatggcgtgaacccgggaggtggagcttgcagtgagccgagattgcgccactgcactccagcctgggcgacagagcgggactccgtctcaaaaaaaaaaaaaaaaagaaattacctttagaattggtaaactacatgagaaaattaagcatattattcatatcttagtgttattacccaacttcatctccaatactttcccctttccctagctagatatgtttttgtttgtttgttttagacagtcttgctctgtcgctcaggctggagtgcaaaggcacgatcttggctcactgcaacctctgcctcgcaggttaaagcgattctcatgtctcagcctcctgcgtagctgggattacaggtgtacaccactgcacccagctaatttttttttttttttttttttaagtatcgacagggtttcaccatgttggccaggctggtctcaaactcctgacctcaagtgatctgcccacctcggcctcccaaagtgttgggattacaggcgtgagccaccatgcctggcctagatattttttattctttccaaaatttaattctccctgaagttaaaaattttcattactgagaatgtacatagagatgtgtcacaaccctttagtaattccaaaaggtgtttcaaaaattttatacaatgataatcactgttgaaacaggtgtatattctcctcagatcatgactgaccaagatgatattccaagaagtaaactactggcctttatagagtaggatgtaggccattttcattactgataacatacttttaaaagaaatgtttacagatttaaataagttaaaacatctaaatgcttttaaaagagcacctggcacattgcaagttattcattattaattagtagatgaatcatatatctggagtgcacccttgctctatatgaaagcttccctaactatagatatataggtgatagactgacaataaagatttgaggaaagaaaaattatttggctggcttattttttaagcttttgagatgtataaggtagagattgtttatcaaataatttatgtgacacattcaatgcatatgaaataattatctaatactgaatttattcaaggactgaaagtatatagagcacacaggctgcaaaccaggaaaactaccagttagagacagggctttattcttggaataaaggtacaatgtaaagagtagatgtttcatgacttgattaaattatttaaaactgtctagaattgtgttataaaactattactatgtttctatgcacttagttattacatgggtttaaatttggcactgtttctaagtttctataaggctttgttgttaagatctttctattcaaaacattaattttaacaaaaagcttttccccgttatttttctgcaactggacttttttgtattactttcctatattaaaacgcatttaaaata

SEQ ID NO: 2 - DNA, 5821 bp, Homo sapiens
ggttccggcccagccatggcggacgaggccccgcggaagggcagcttctcggcgctcgtgggccgcaccaacggcctcaccaagcccgcggccctggccgccgcgcccgccaagccggggggcgcgggcggctccaagaagctggtcatcaagaacttccgagacagacctcggctgcccgacaactacacgcaggacacgtggcggaagctgcacgaggcggtgcgggccgtgcagagcagcacctccatcaggtacaacctcgaggagctctaccaggctgtggaaaatctctgttctcacaaagtctccccaatgctctacaagcaactgcgtcaggcctgtgaagaccacgtccaggcacagatccttccgtttagagaagactcactagatagtgttttatttttaaagaagattaacacgtgctggcaggaccactgcagacaaatgatcatgatcagaagcatcttcctgttcttggaccgcacctatgtgctgcagaactccacgctgccctccatctgggatatgggattagaactgtttagaacccatattattagtgataaaatggttcagagtaaaaccattgatggaatcctactgctgatcgagcgcgagaggagcggcgaggccgtggaccggagcctgttgcggagcctcctgggcatgctgtctgacctgcaggtgtataaagattcatttgaactgaaatttttggaagagactaattgcttatatgctgccgaaggccaaaggttaatgcaggaaagagaggttccagaatatcttaaccatgtaagtaaacgcttagaggaagagggagacagagtaatcacttacttggaccacagcacacagaaaccactgattgcttgtgtggagaaacagctattaggagaacatttaacagcaattctgcagaaagggctcgaccacttactggatgagaacagagtgccggacctcgcacagatgtaccagctgttcagccgggtgaggggcgggcagcaggcgctgctgcagcactggagcgagtacatcaagacttttggaacagcgatcgtaatcaatcctgagaaagacaaagacatggtccaagacctgttggacttcaaggacaaggtggaccacgtgatcgaggtctgcttccagaagaatgagcggttcgtcaacctgatgaaggagtcctttgagacgttcatcaacaagagacccaacaagcctgcagaactgatcgcaaagcatgtggattcaaagttaagagcaggcaacaaagaagccacagacgaggagctggagcggacgttggacaagatcatgatcctgttcaggtttatccacggtaaagatgtctttgaagcattttataaaaaagatttggcaaaaagactccttgttgggaaaagtgcctcagtcgatgctgaaaagtctatgttgtcaaagctcaagcatgagtgcggtgcagccttcaccagcaagctggaaggcatgttcaaggacatggagctttcgaaggacatcatggttcatttcaagcagcatatgcagaatcagagtgactcaggccctatagacctcacagtgaacatactcacaatgggctactggccaacatacacgcccatggaagtgcacttaaccccagaaatgattaaacttcaggaagtatttaaggcattttatcttggaaagcacagtggtcgaaaacttcagtggcaaactactttgggacatgctgttttaaaagcggagtttaaagaagggaagaaggaattccaggtgtccctcttccagacactggtgctcctcatgttcaacgagggagatggcttcagctttgaggagataaaaatggccacggggatagaggatagtgaattgcgcagaacgctgcagtccctggcctgtggcaaagcacgtgtgctgattaaaagtcccaaaggaaaggaagtggaagatggagacaagttcatttttaatggagagttcaagcacaagttgtttagaataaagatcaatcaaattcagatgaaggaaactgttgaggaacaggttagcaccactgagagagtgtttcaggatagacaatatcagattgatgctgctatcgtcagaataatgaagatgagaaagactcttggtcataatcttctagtttctgaattatataatcagctgaaatttccagtaaagcctggagatttgaaaaagagaattgaatctctgatagacagagactatatggagagagacaaagacaatccgaatcagtaccactacgtggcctgacgcatctgcagacggttccccttcatgaaacactagaatgtaccctcagagcaggaagcacacctgtgccatttctgggactctgattgatccagctgtggacattggaaggcgaaggaagggaggtggctcctgggtcatctttcacaaggctcaagacttcaacctgcagatgtatctttttccctccagtttttcctctagttcttttaggcatttaaattgtttctgttactctgtgcaaaataactttgagattggacaagaagatgttactaaagagaagttcctttaaaaggtcttgttcttgtgtcaaaaagctgcaagtttggtttgttctcgtgtgtgatcatgagtgcacaatgaagaagaccctagatgctgcattttttagctctgaagattccttaggtatccctgaagacagctcgctcagatgatcagcatttagagtgaaaacaagggcccttcatgggtgaacattagaaagagccagggttcaaagctggcgaatggatgacgcaccctagccactggcccctctctgtttcatgtatttccaaaagttgtaaactttgatggctgatttttcgtaagtcaggtttctaagtgagctccctgaggtgccaaggccatggtgtccgccctgctgcgtctgttcgtcagctgagttccttgtgaatctctgttttagggtttggggctagtgtgtttgtgtttccattctaagattgagtctggcagtccctgtttttttgcattggggtaactgctctttgattttttttaattgcagtatttgtgtgattgcaataataaagtttggtttggtttttacagtcatgcgcagggacgatccttgttctctgctgtaaactgtaaaaagtttatggagacttaaagtcttgatgttgtgaagcagaggttattttgtggaaagattaaaaggattttgttggtacctggttttgtgttgtgtatatatacatgaggttgaacagtgaaaggaaagttcagtagtgatgttagaagggtaactatgacaaagatacttttgagataacatttaaaagtactttatattttacataatagcatgtttcattttgattaaaagctaccaaaggaattttgatcatggcataagtgtttaaagcaatattttctggaatataccaagtttatataatttgattttgtgctaaattattaagagtctctttttgaaacatgcgggtttgaaatatgacaccttgtgggtttccatattaaaatcctcactctttaattgtcatttctatctttgaaaattttcatttatgagttccatgatatgtggtctaagaaagaccaaacagatttctattttttttttcttataagttcgttgtgtctagagattgttaatattgtaatttaatgtagacttactttgaataaaattagtttaattggccttaaaattacattaataaaactttgtgatatgcaaatgacacattcttcataactctttagcagctttgactactagtgcactagacagaagtcagagcagggagcacctgtcccctctcaagtgattattctttcctggccacctctaccacaaaataccagtggggccaggtagtgacaagtgggtcttttttacttggacgattcgttgtgctgtgcctttgtttcatttgagcacagtggctcacgcctgtagtcccagctatgggagggcaaggtgggaggatcgtttgagcctgagttccagaccatcctgagcaccatagggagatcctgtttccattttagtttatttatttttaattgaggtggagtcttgctctgttgcccaagctggagtgcagtggtgcaatctcagctcactgcaccctccgcctcctgggttcaagcagttctcccacctcagtctcccaagtagctgggattacaggcacccgccatcatgcccagctaatatttgtatttttgtagagacggggtttcactatgttggccagactggtcttgaactcctaacctcaggtgatctgcccgccttggcctcccaaagtgctgggattacaggcgtgagccaccatgcccggcctgcctgtttctgttttataaaagaaaggaaaatctatttatatctattctcttatttagcaatatttaatgttttattgttaaaggtcagtgtggtaaaacaaatagtatagaagaaatcattgaaaaagaaacagcacttagacagaaatgctgtaaaagtggaaaggagaaggtgaaattacttgcaggttagatggttgcatacccaggtcatctaaggagcaaatgaaaatctgtgactgaagaaagaattcaccaagttaaccagacacaaaattaacaaaaacatcagtagctttcctataaatataggctataatggagggtcattttttatttttatttagagacagggtcttaactgtcacctggactggagtgcagtggcatgatcatgtttcacggcagcctctaccttctgggctcaagcgatcctctcttctcagccacctgagtagctgggcctacaggtgtacatcaccacgcccagataatttttattgtattttttatagaggcagtgtcttgctatgttgccaaggctgttcttgtactcctggcctcaagcgaacctcctacctcagcctccccaaatgctgggattacaggcatgagacactgcacctgaccagaagtcattttttcaatagcaacccccaaaaaagataaaatacctagtaacaaatagggaaacacctatgtgaaaggtattataacattactaaggaacacaggccctgaataagtgaaagttctgttgattctcacattttgctatacagtatcttaagatgtaaaaccttcctttaaaacacaagcggattctaaagttaaaacagaaaagcaaatatgccagactagtcaaattgttttaaattctgctgtttttagaacattgtaattgaaacagcatgatgctggccctttaaaaagattcctggaacaagaaagtccacaaataagccaaatacacaggaactcggcgtggcacaaaggggccgtgtgtgatcaggaactggaactttgcaacaactacccatgctcagaagtttgggccaccttgaaaagagaaaagttggattagactcctttttatactaagggaagttccaagtggtcaagtatttacgtgtaaaaaaatacatatatatgaaaccataatcataagatactttttttgtaaattgactattattgtataaatttatagagtataaagtgatcttataaattatgcatacattgtggactagtcaagctagttacatccatcacctcaaatacttaacatttttgtagtgagaacatctgaaatttactcttagcaattttgaaatgtacaatactcaatttttgactgtattcaccatgctgtacaatagaactcagaaaaagaaaaatatagtcctcctttctaaga

SEQ ID NO: 3 - DNA, 3719 bp, Homo sapiens
gccgagccgggactgcgctagcccgccgcgctctgggctgcccgagcgagcgttcggacctcgcaccccgcgcgccccgcgccgccgccgccgccggcttttgttgtctccgcctcctcggccgccgccgcctctggaccgcgagccgcgcgcgccgggaccttggctctgcccttcgcgggcgggaactgcgcaggacccggccaggatccgagagaggcgcgggcgggtggccgggggcgccgccggccccgccatggagctccgggcccgaggctggtggctgctatgtgcggccgcagcgctggtcgcctgcgcccgcggggacccggccagcaagagccggagctgcggcgaggtccgccagatctacggagccaagggcttcagcctgagcgacgtgccccaggcggagatctcgggtgagcacctgcggatctgtccccagggctacacctgctgcaccagcgagatggaggagaacctggccaaccgcagccatgccgagctggagaccgcgctccgggacagcagccgcgtcctgcaggccatgcttgccacccagctgcgcagcttcgatgaccacttccagcacctgctgaacgactcggagcggacgctgcaggccaccttccccggcgccttcggagagctgtacacgcagaacgcgagggccttccgggacctgtactcagagctgcgcctgtactaccgcggtgccaacctgcacctggaggagacgctggccgagttctgggcccgcctgctcgagcgcctcttcaagcagctgcacccccagctgctgctgcctgatgactacctggactgcctgggcaagcaggccgaggcgctgcggcccttcggggaggccccgagagagctgcgcctgcgggccacccgtgccttcgtggctgctcgctcctttgtgcagggcctgggcgtggccagcgacgtggtccggaaagtggctcaggtccccctgggcccggagtgctcgagagctgtcatgaagctggtctactgtgctcactgcctgggagtccccggcgccaggccctgccctgactattgccgaaatgtgctcaagggctgccttgccaaccaggccgacctggacgccgagtggaggaacctcctggactccatggtgctcatcaccgacaagttctggggtacatcgggtgtggagagtgtcatcggcagcgtgcacacgtggctggcggaggccatcaacgccctccaggacaacagggacacgctcacggccaaggtcatccagggctgcgggaaccccaaggtcaacccccagggccccgggcctgaggagaagcggcgccggggcaagctggccccgcgggagaggccaccttcaggcacgctggagaagctggtctccgaagccaaggcccagctccgcgacgtccaggacttctggatcagcctcccagggacactgtgcagtgagaagatggccctgagcactgccagtgatgaccgctgctggaacgggatggccagaggccggtacctccccgaggtcatgggtgacggcctggccaaccagatcaacaaccccgaggtggaggtggacatcaccaagccggacatgaccatccggcagcagatcatgcagctgaagatcatgaccaaccggctgcgcagcgcctacaacggcaacgacgtggacttccaggacgccagtgacgacggcagcggctcgggcagcggtgatggctgtctggatgacctctgcagccggaaggtcagcaggaagagctccagctcccggacgcccttgacccatgccctcccaggcctgtcagagcaggaaggacagaagacctcggctgccagctgcccccagcccccgaccttcctcctgcccctcctcctcttcctggcccttacagtagccaggccccggtggcggtaactgccccaaggccccagggacagaggccaaggactgactttgccaaaaatacaacacagacgatatttaattcacctcagcctggagaggcctggggtgggacagggagggccggcggctctgagcaggggcaggcgcagaggtcccagccccaggcctggcctcgcctgcctttctgccttttaattttgtatgaggtcctcaggtcagctgggagccagtgtgcccaaaagccatgtatttcagggacctcaggggcacctccggctgcctagccctccccccagctccctgcaccgccgcagaagcagcccctcgaggcctacagaggaggcctcaaagcaacccgctggagcccacagcgagcctgtgccttcctccccgcctcctcccactgggactcccagcagagcccaccagccagccctggcccaccccccagcctccagagaagccccgcacgggctgtctgggtgtccgccatccagggtctggcagagcctctgagatgatgcatgatgccctcccctcagcgcaggctgcagagcccggccccacctccctgcgcccttgaggggccccagcgtctgcagggtgacgcctgagacagcaccactgctgaggagtctgaggactgtcctcccacagacctgcagtgaggggccctccatgcgcagatgaggggccactgacccacctgcgcttctgctggaggaggggaagctgggcccaaaggcccagggaggcagcgtgggctctgccaatgtgggctgcccctcgcacacagggctcacagggcaggccttgctggggtccagggctgttggaggaccccgagggctgaggagcagccaggacccgcctgctcccatcctcacccagatcaggaaccagggcctccctgttcacggtgacacaggtcagggctcagagtgaccctcagctgtcacctgctcacagggatgctggtggctggtgagaccccgcactgcagacgggaatgcctaggtcccttcccgacccagccagctgcagggcacggggacctggatagttaagggcttttccaaacatgcatccatttactgacacttcctgtccttgttcatggagagctgttcgctcctcccagatggcttcggagggccgcagggcccaccttggaccctggtgacctcctgtcactcactgaggccatcagggccctgccccaggcctggacgggccctccttccctcctgtgccccagctgccaggcggccctggggaggggtggtgtggtgttgggaaggggtcctgcagggggaggaggacttggagggtctgggggcagctgtcctgaaccgactgaccctgaggaggccgcttagtgctgctttgcttttcatcaccgtcccgcacagtggacggaggtccccggttgctggtcaggtccccatggcttgttctctggaacctgactttagatgttttgggatcaggagcccccaacacaggcaagtccaccccataataaccctgccagtgccagggtgggctggggactctggcacagtgatgccgggcgccaggacagcagcactcccgctgcacacagacggcctaggggtggcgctcagaccccaccctacgctcatctctggaaggggcagccctgagtggtcactggtcagggcagtggccaagcctgctgtgtccttcctccacaaggtccccccaccgctcagtgtcagcgggtgacgtgtgttcttttgagtccttgtatgaataaaaggctggaaaccta

SEQ ID NO: 4 - DNA, 1923 bp, Homo sapiens
gagacgaaacttcccgtcccggcggctctggcacccagggtccggcctgcgccttcccgccaggcctggacactggttcaacacctgtgacttcatgtgtgcgcgccggccacacctgcagtcacacctgtagccccctctgccaagagatccataccgaggcagcgtcggtggctacaagccctcagtccacacctgtggacacctgtgacacctggccacacgacctgtggccgcggcctggcgtctgctgcgacaggagcccttacctcccctgttataacacctgaccgccacctaactgcccctgcagaaggagcaatggccttggctcctgagagggcagccccacgcgtgctgttcggagagtggctccttggagagatcagcagcggctgctatgaggggctgcagtggctggacgaggcccgcacctgtttccgcgtgccctggaagcacttcgcgcgcaaggacctgagcgaggccgacgcgcgcatcttcaaggcctgggctgtggcccgcggcaggtggccgcctagcagcaggggaggtggcccgccccccgaggctgagactgcggagcgcgccggctggaaaaccaacttccgctgcgcactgcgcagcacgcgtcgcttcgtgatgctgcgggataactcgggggacccggccgacccgcacaaggtgtacgcgctcagccgggagctgtgctggcgagaaggcccaggcacggaccagactgaggcagaggcccccgcagctgtcccaccaccacagggtgggcccccagggccattcctggcacacacacatgctggactccaagccccaggccccctccctgccccagctggtgacaagggggacctcctgctccaggcagtgcaacagagctgcctggcagaccatctgctgacagcgtcatggggggcagatccagtcccaaccaaggctcctggagagggacaagaagggcttcccctgactggggcctgtgctggaggcccagggctccctgctggggagctgtacgggtgggcagtagagacgacccccagccccgggccccagcccgcggcactaacgacaggcgaggccgcggccccagagtccccgcaccaggcagagccgtacctgtcaccctccccaagcgcctgcaccgcggtgcaagagcccagcccaggggcgctggacgtgaccatcatgtacaagggccgcacggtgctgcagaaggtggtgggacacccgagctgcacgttcctatacggccccccagacccagctgtccgggccacagacccccagcaggtagcattccccagccctgccgagctcccggaccagaagcagctgcgctacacggaggaactgctgcggcacgtggcccctgggttgcacctggagcttcgggggccacagctgtgggcccggcgcatgggcaagtgcaaggtgtactgggaggtgggcggacccccaggctccgccagcccctccaccccagcctgcctgctgcctcggaactgtgacacccccatcttcgacttcagagtcttcttccaagagctggtggaattccgggcacggcagcgccgtggctccccacgctataccatctacctgggcttcgggcaggacctgtcagctgggaggcccaaggagaagagcctggtcctggtgaagctggaaccctggctgtgccgagtgcacctagagggcacgcagcgtgagggtgtgtcttccctggatagcagcagcctcagcctctgcctgtccagcgccaacagcctctatgacgacatcgagtgcttccttatggagctggagcagcccgcctagaacccagtctaatgagaactccagaaagctggagcagcccacctagagctggccgcggccgcccagtctaataaaaagaactccagaaca

SEQ ID NO: 5 - DNA, 3068 bp, Homo sapiens
gcgccggggtggagtcatcctgggaacctccacgcgactttggtggaggtagttctttggcagcgggcatggcgggtaccgtggtgctggacgatgtggagctgcgggaggctcagagagattacctggacttcctggacgacgaggaagaccagggaatttatcagagcaaagttcgggagctgatcagtgacaaccaataccggctgattgtcaatgtgaatgacctgcgcaggaaaaacgagaagagggctaaccggcttctgaacaatgcctttgaggagctggttgccttccagcgggccttaaaggattttgtggcctccattgatgctacctatgccaagcagtatgaggagttctacgtaggactggaaggcagctttggctccaagcacgtctccccgcggactcttacctcctgcttcctcagctgtgtggtctgtgtggagggcattgtcactaaatgttctctagttcgtcccaaagtcgtccgcagtgtccactactgtcctgctactaagaagaccatagagcgacgttattctgatctcaccaccctggtggcctttccctccagctctgtctatcctaccaaggatgaggagaacaatccccttgagacagaatatggcctttctgtctacaaggatcaccagaccatcaccatccaggagatgccggagaaggccccagccggccagctcccccgctctgtggacgtcattctggatgatgacttggtggataaagcgaagcctggtgaccgggttcaggtggtgggaacctaccgttgccttcctggaaagaagggaggctacacctctgggaccttcaggactgtcctgattgcctgtaatgttaagcagatgagcaaggatgctcagccctctttctctgctgaggatatagccaagatcaagaagttcagtaaaacccgatccaaggatatctttgaccagctggccaagtcattggccccaagtatccatgggcatgactatgtcaagaaagcaatcctctgcttgctcttgggaggggtggaacgagacctagaaaatggcagccacatccgtggggacatcaatattcttctaataggagacccatccgttgccaagtctcagcttctgcggtatgtgctttgcactgcaccccgagctatccccaccactggccggggctcctctggagtgggtctgacggctgctgtcaccacagaccaggaaacaggagagcgccgtctggaagcaggggccatggtcctggctgaccgaggcgtggtttgcattgatgaatttgacaaaatgtctgacatggatcgcacagccatccatgaagtgatggagcagggtcgagtgaccattgccaaggctggcatccatgctcggctgaatgcccgctgcagtgttttggcagctgccaaccctgtctacggcaggtatgaccagtataagactccaatggagaacattgggctacaggactcactgctgtcacgatttgacttgctcttcatcatgctggatcagatggatcctgagcaggatcgggagatctcagaccatgtccttcggatgcaccgttacagagcacctggggagcaggatggcgatgctatgcccttgggtagtgctgtggatatcctggccacagatgatcccaactttagccaggaagatcagcaggacacccagatttatgagaagcatgacaaccttctacatgggaccaagaagaaaaaggagaagatggtgagtgcagcattcatgaagaagtacatccatgtggccaaaatcatcaagcctgtcctgacacaggagtcggccacctacattgcagaagagtattcacgcctgcgcagccaggatagcatgagctcagacaccgccaggacatctccagttacagcccgaacactggaaactctgattcgactggccacagcccatgcgaaggcccgcatgagcaagactgtggacctgcaggatgcagaggaagctgtggagttggtccagtatgcttactttaagaaggttctggagaaggagaagaaacgtaagaagcgaagtgaggatgaatcagagacagaagatgaagaggagaaaagccaagaggaccaggagcagaagaggaagagaaggaagactcgccagccagatgccaaagatggggattcatacgacccctatgacttcagtgacacagaggaggaaatgcctcaagtacacactccaaagacggcagactcacaggagaccaaggaatcccagaaagtggagttgagtgaatccaggttgaaggcattcaaggtggccctcttggatgtgttccgggaagctcatgcgcagtcaatcggcatgaatcgcctcacagaatccatcaaccgggacagcgaagagcccttctcttcagttgagatccaggctgctctgagcaagatgcaggatgacaatcaggtcatggtgtctgagggcatcatcttcctcatctgaggaggcctcgtctctgaacttgggttgtgccgagagagtttgttctgtgtttcccaccctctccctgacccaagtctttgcctctactcccttaacagtgttgaattcaactgaaggcgaggaatgttggtgatgaagctgagttcaggactcggtggaccctttgggaatgggtcatgaaagctgccatggggtgaggaaagaggagacagtgggagaggacaatgactattgcatcttcattgcaaaagcactggctcatccgccctacttcccatcccacacaaacccaattgtaaataacatatgacttctgagtacttttgggggcacaactgttttctgtttgctgtttttttgttttgttttttttctccagagcactttggtctagactaggctttgggtggttccaattggtggagagaagctctgaggcacgtcatgcaggtcaagaaagctttctttgcagtagcaccagttaaggtgaatatgtattgtatcacaaaacaaacccaatatccagatgaatatccgagatgttgaataaacttagccatttcgtacacatgg

SEQ ID NO: 6 - DNA, 6411 bp, Homo sapiens
aaagggggcggcagcgccggcggagcggaggcgggtctcacgtgggccagcgcagagcctgcggaagggacggatgcggatctcgtcgctgtcaccttgaaagtgaccgaggggcttgactgtggactccttacgccgcccacccgggcccggcggtcccagccttctcgcagggccccttctcagcagaagcaagcggggccgagaaagcgggtggaatagggttgctgcaggtcccaaagacccctcgtggcgcctcgctactttctgcagcttgtttgcactttttcacgctctagaaaaatctcatcttaattaagggaacaacaaatcatttaatcttcagagcatcttagactgaaaacctttcaactgtgctgaaaaacctagaagacagaccattttgcccaccctctcatttaaaaggaattgaagaagaaataaaatggcagaggtttaaggttactattcaggatgactgatgataattcagatgataaaatagaagatgaattgcaaaccttctttaccagtgataaagatggaaatacacatgcatacaacccgaaatcaccacctacacaaaactcttcagccagcagtgtgaactggaattctgccaacccagatgacatggtggttgattatgaaactgaccctgctgtagttactggtgaaaatatttctttaagccttcagggtgttgaagtatttggtcatgaaaagtcttctagtgatttcattagtaagcaggtgttagatatgcataaagattctatttgtcagtgtcctgcacttgtaggtactgagaagcccaaatatctgcaacacagttgtcattccctagaagcagttgagggccagagtgttgagccatctttgccttttgtgtggaagcctaatgacaatttgaactgtgcaggctactgtgatgccttggagctaaaccaaacatttgacatgacagtggataaagttaactgcacctttatatcacatcatgccatcggaaagagtcagtccttccatactgctggaagcctgccaccaactggtaggagaagtggaagtacatcttctttatcctattccacttggacatcttcccattctgataagacgcatgcaagagaaactacttatgatagagaaagctttgaaaaccctcaagtcacaccatcagaagcccaagacatgacttacacagcattttctgatgtggtgatgcaaagtgaggtttttgtttcagatattggaaatcagtgtgcatgttcttcaggaaaggtcaccagtgagtacacagatggatcacaacaaagactagttggagaaaaggagacacaagcactaacaccagtttctgatggcatggaagtccccaatgattctgcattacaagagttcttttgtttatcccatgatgaatccaatagcgaaccacattcacagagctcatacaggcacaaggaaatgggccaaaatctgagagagacagtgtcctattgtcttattgatgatgaatgccctttaatggtgccagcttttgataagagcgaagctcaagtgctgaacccagagcataaagtcactgagactgaagacacacaaatggtctccaaaggaaaggatttgggaacccaaaatcatacctcagaattgattctaagtagcccgccaggacaaaaggtgggctcgtcatttggactgacttgggatgcaaatgatatggtcattagcacagacaaaacgatgtgcatgtcaacaccagtcctagaacccacaaaagtaaccttttctgtttcaccgattgaagcgacggagaaatgtaagaaagtggagaagggtaatcgagggcttaaaaacataccagactcgaaggaggcacctgtgaacctgtgtaaacccagtttaggaaaatcaacaatcaaaacgaataccccaataggctgcaaagttagaaaaactgaaattataagttacccaagaccaaacttcaagaatgtcaaagcaaaagttatgtctagagcagtgttgcagcccaaagatgctgctttatcaaaggtcacgcccagacctcagcagaccagtgcctcatcaccctcatcagtgaattcaagacaacaaacagtcttgagcagaacaccgagatctgacttgaatgcagacaaaaaagcagaaattctaattaacaagacacataagcagcagtttaataaactcattactagccaggctgtgcatgttacaactcattctaaaaatgcttcacacagggttccaagaacaacatctgccgtgaaatcgaatcaggaagatgttgacaaagccagttcttctaactcagcatgcgagaccgggtccgtttctgcgttgtttcagaagatcaaaggcatactccctgttaaaatggaaagtgcagaatgtttggaaatgacctatgttcccaacattgataggattagccctgaaaagaagggtgaaaaagaaaatgggacatctatggaaaaacaagagctgaaacaagagattatgaatgagacttttgaatatggttctctgtttttgggctctgcttcaaaaacaacgaccacctcaggtaggaatatatccaagcctgactcctgcggtttgaggcaaatagctgctccaaaagccaaagtggggccccctgtttcctgtttgaggcggaacagtgacaatagaaatcccagtgctgatcgagccgtatctcctcagaggatcaggcgtgtgtccagttctggaaagcctacatccttgaaaactgcacagtcgtcatgggtgaatttgcctagaccacttcctaaatccaaagcatctttgaaaagtcctgcgctgcggaggacaggaagcaccccctcaatagccagcacccacagtgagctgagcacttacagcaacaattctggtaatgccgctgtcatcaaatatgaggagaaacctccaaaaccagcatttcagaatggttcctcaggatccttttatttgaagcctttggtatccagggctcatgttcacttgatgaaaactcctccaaaaggtccttcgagaaaaaatttatttacagctcttaatgcagttgaaaagagcaggcaaaagaatcctcgaagcttatgtatccagccacagacagctcccgatgcgctgccccctgagaaaacacttgaattgacgcaatataaaacaaaatgtgaaaaccaaagtggatttatcctgcagctcaagcagcttcttgcctgtggtaataccaagtttgaggcattgacagttgtgattcagcacctgctgtctgagcgggaggaagcactgaaacaacacaaaaccctatctcaagaacttgttaacctccggggagagctagtcactgcttcaaccacctgtgagaaattagaaaaagccaggaatgagttacaaacagtgtatgaagcattcgtccagcagcaccaggctgaaaaaacagaacgagagaatcggcttaaagagttttacaccagggagtatgaaaagcttcgggacacttacattgaagaagcagagaagtacaaaatgcaattgcaagagcagtttgacaacttaaatgctgcgcatgaaacctctaagttggaaattgaagctagccactcagagaaacttgaattgctaaagaaggcctatgaagcctccctttcagaaattaagaaaggccatgaaatagaaaagaaatcgcttgaagatttactttctgagaagcaggaatcgctagagaagcaaatcaatgatctgaagagtgaaaatgatgctttaaatgaaaaattgaaatcagaagaacaaaaaagaagagcaagagaaaaagcaaatttgaaaaatcctcagatcatgtatctagaacaggagttagaaagcctgaaagctgtgttagagatcaagaatgagaaactgcatcaacaggacatcaagttaatgaaaatggagaaactggtggacaacaacacagcattggttgacaaattgaagcgtttccagcaggagaatgaagaattgaaagctcggatggacaagcacatggcaatctcaaggcagctttccacggagcaggctgttctgcaagagtcgctggagaaggagtcgaaagtcaacaagcgactctctatggaaaacgaggagcttctgtggaaactgcacaatggggacctgtgtagccccaagagatcccccacatcctccgccatccctttgcagtcaccaaggaattcgggctccttccctagccccagcatttcacccagatgacacctccccaaagtccacagactctctgaaagcattttgatgcaggtctgcaggactgaccccaaggaggaacgtgggcacaagaggtatatcagcacacgtgtgatcaccgtagggtaactggagcgtcaccaccggcggaatcgcagcttctgagactggaactctggaggaagacttttgcctccgtccaaaagattcctccaaaaaaagatttaaaaaaagatttcggcatcgacacggacgttgttgcacaaagcacttaaagaacgagagcatcttgttcattgcctttttcacctaagcatagggggaaaaactctcagggccctattaagatttataacctttgtaatgttcttcaccacagacaccttcttgtgagttttcagtctgactgtgggggtggggggtgtgaatgaaatggatgtcacagagtgtcatgtgtctgatgcagcctcctctgctgtgtattaaatgtcaaaatctgaatatatctggatatgtactaatcaaataataatcaatcaatcagcatatacatttcagccaaagccatagaagaaaaagcaatagttgcttgaattatgatcatctaccaccaactctgctcagccctgtaacagggtagggagagggtataacaggaagagctttgacttgtccctgtctatacattctctgtatcttttgggggtaacttcttggcagtttttcagtgttcagccatgtcagttgaaactagatttttctgtagattttttacttacccatgtgagcctaacactatcctgtaattcattttctcaggctatgtgtaaatgtagaaccctaatttttctataaaaaaacaaactaactaactaactgtgtaaagaaagaaaaagggaagtaccaatgggtttttccaccttatttttacctttgatctacccttgcagatttaacctgtcttcttccctcccattattctcattttccttttacctttctccaccatccagagccacaaaagcaaaccttctacctcctacctacttttctctgggacaaggataaaggaatatgattttccagagccccagagccagctcatcttccaggtgctgaaaccactttccaaataaactaaagcctggatttgatattacaaattttgggaaatcttagaataaagaacgagaacaaggaagtcattggctagtataattaagaaaggtaggattcagtgcttaccgatgatgcagtacttgatagaagaaaacagtctgggaggatagcgctcatttttcagttaccctttaaggagtccctttgtctttgggaaagtagcagaatggtccgcttctttcccatgagtggaaaatgtggcttgtccaactctcctccaggttgcatttcagtttctttccaaaacttattacctcccctaatcctgagactttggaaaaggtggaaggaagaactgttgctttatctccccctccctgcatgtgtcaacattgtgatgtcagtatttactaatctacattcagtggctgtacaaataacagctgtagtaagaagagattcaggatgctagaggtgaatatttgggtcatttacatgtacactacatagcaagttgatactcatgttgcatgttcttttaaattagtgattttgtgtcttaagtctttaacttccaatacttcatcatgtatgtaaccttccatgtttgcttctgataaatggaaatgtaggttcactgccacttcatgagatatctctgctcacgcttccaagttgttctcaatgacattagccaaagttgggtttgccattcatcccctaggcatggtaaatcttgtgttgttccctgctgtcctccgtattacgtgaccggcaaataaatctcatagcagttaatataaaacatctttggaggatgggagagaacaggagggaagatgggaaacaaaatagagaattcttaagattttgtttaaaccaaatgtttcatgtagaatgcaaaatgttggcacgtcaaaaatatgaatgtgtagacaactgtagttgtgctcagtttgtagtgatgggaagtgtattttactctgatcaaataaataatgctggaatactcaa

SEQ ID NO: 7 - DNA, 1355 bp, Homo sapiens
ggatggccggagctggcgccctggttctggaggtaaccggttactgagggcgagaagcgccacccggaggctctagcctgacaaatgcttgctgacctgggccagagctcttcccttacgcaagtctcagccggtcgtcgcgacgttcgcccgctcgctctgaggctcctgaagccgaaaccagctagactttcctccttcccgcctgcctgtagcggcgttgttgccactccgccaccatgttcgaggcgcgcctggtccagggctccatcctcaagaaggtgttggaggcactcaaggacctcatcaacgaggcctgctgggatattagctccagcggtgtaaacctgcagagcatggactcgtcccacgtctctttggtgcagctcaccctgcggtctgagggcttcgacacctaccgctgcgaccgcaacctggccatgggcgtgaacctcaccagtatgtccaaaatactaaaatgcgccggcaatgaagatatcattacactaagggccgaagataacgcggataccttggcgctagtatttgaagcaccaaaccaggagaaagtttcagactatgaaatgaagttgatggatttagatgttgaacaacttggaattccagaacaggagtacagctgtgtagtaaagatgccttctggtgaatttgcacgtatatgccgagatctcagccatattggagatgctgttgtaatttcctgtgcaaaagacggagtgaaattttctgcaagtggagaacttggaaatggaaacattaaattgtcacagacaagtaatgtcgataaagaggaggaagctgttaccatagagatgaatgaaccagttcaactaacttttgcactgaggtacctgaacttctttacaaaagccactccactctcttcaacggtgacactcagtatgtctgcagatgtaccccttgttgtagagtataaaattgcggatatgggacacttaaaatactacttggctcccaagatcgaggatgaagaaggatcttaggcattcttaaaattcaagaaaataaaactaagctctttgagaactgcttctaagatgccagcatatactgaagtcttttctgtcaccaaatttgtacctctaagtacatatgtagatattgttttctgtaaataacctatttttttctctattctctgcaatttgtttaaagaataaagtccaaagtcagatctggtctagttaacctagaagtatttttgtctcttagaaatacttgtgatttttataatacaaaagggtcttgactctaaatgcagttttaagaattgtttttgaatttaaataaagttacttgaatttcaaacatca

SEQ ID NO: 8 - DNA, 3786 bp, Homo sapiens
aggttcaaacacagacggcgggtgaacatggcgtcctcgacttggtctgagacgtgataggcctgccttctggttgaagatgtggcgagtgaaaaaactgagcctcagcctgtcgccttcgccccagacgggaaaaccatctatgagaactcctctccgtgaacttaccctgcagcccggtgccctcaccaactctggaaaaagatcccccgcttgctcctcgctgaccccatcactgtgcaagctggggctgcaggaaggcagcaacaactcatctccagtggattttgtaaataacaagaggacagacttatcttcagaacatttcagtcattcctcaaagtggctagaaacttgtcagcatgaatcagatgagcagcctctagatccaattccccaaattagctctactcctaaaacgtctgaggaagcagtagacccactgggcaattatatggttaaaaccatcgtccttgtaccatctccactggggcagcaacaagacatgatatttgaggcccgtttagataccatggcagagacaaacagcatatctttaaatggacctttgagaacagacgatctggtgagagaggaggtggcaccctgcatgggagacaggttttcagaagttgctgctgtatctgagaaacctatctttcaggaatctccgtcccatctcttagaggagtctccaccaaatccctgttctgaacaactacattgctccaaggaaagcctgagcagtagaactgaggctgtgcgtgaggacttagtaccttctgaaagtaacgccttcttgccttcctctgttctctggctttccccttcaactgccttggcagcagatttccgtgtcaatcatgtggacccagaggaggaaattgtagagcatggagctatggaggaaagagaaatgaggtttcccacacatcctaaggagtctgaaacagaagatcaagcacttgtctcaagtgtggaagatattctgtccacatgcctgacaccaaatctagtagaaatggaatcccaagaagctccaggcccagcagtagaagatgttggtaggattcttggctctgatacagagtcttggatgtccccactggcctggctggaaaaaggtgtaaatacctccgtcatgctggaaaatctccgccaaagcttatcccttccctcgatgcttcgggatgctgcaattggcactacccctttctctacttgctcggtggggacttggtttactccttcagcaccacaggaaaagagtacaaacacatcccagacaggcctggttggcaccaagcacagtacttctgagacagagcagctcctgtgtggccggcctccagatctgactgccttgtctcgacatgacttggaagataacctgctgagctctcttgtcattctggaggttctctcccgccagcttcgggactggaagagccagctggctgtccctcacccagaaacccaggacagtagcacacagactgacacatctcacagtgggataactaataaacttcagcatcttaaggagagccatgagatgggacaggccctacagcaggccagaaatgtcatgcaatcatgggtgcttatctctaaagagctgatatccttgcttcacctatccctgttgcatttagaagaagataagactactgtgagtcaggagtctcggcgtgcagaaacattggtctgttgctgttttgatttgctgaagaaattgagggcaaagctccagagcctcaaagcagaaagggaggaggcaaggcacagagaggaaatggctctcagaggcaaggatgcggcagagatagtgttggaggctttctgtgcacacgccagccagcgcatcagccagctggaacaggacctagcatccatgcgggaattcagaggccttctgaaggatgcccagacccaactggtagggcttcatgccaagcaagaagagctggttcagcagacagtgagtcttacttctaccttgcaacaagactggaggtccatgcaactggattatacaacatggacagctttgctgagtcggtcccgacaactcacagagaaactcacagtcaagagccagcaagccctgcaggaacgtgatgtggcaattgaggaaaagcaggaggtttctagggtgctggaacaagtctctgcccagttagaggagtgcaaaggccaaacagaacaactggagttggaaaacagtcgtctagcaacagatctccgggctcagttgcagattctggccaacatggacagccagctaaaagagctacagagtcagcatacccattgtgcccaggacctggctatgaaggatgagttactctgccagcttacccagagcaatgaggagcaggctgctcaatggcaaaaggaagagatggcactaaaacacatgcaggcagaactgcagcagcaacaagctgtcctggccaaagaggtgcgggacctgaaagagaccttggagtttgcagaccaggagaatcaggttgctcacctggagctgggtcaggttgagtgtcaattgaaaaccacactggaagtgctccgggagcgcagcttgcagtgtgagaacctcaaggacactgtagagaacctaacggctaaactggccagcaccatagcagataaccaggagcaagatctggagaaaacacggcagtactctcaaaagctagggctgctgactgagcaactacagagcctgactctctttctacagacaaaactaaaggagaagactgaacaagagacccttctgctgagtacagcctgtcctcccacccaggaacaccctctgcctaatgacaggaccttcctgggaagcatcttgacagcagtggcagatgaagagccagaatcaactcctgtgcccttgcttggaagtgacaagagtgctttcacccgagtagcatcaatggtttcccttcagcccgcagagaccccaggcatggaggagagcctggcagaaatgagtattatgactactgagcttcagagtctttgttccctgctacaagagtctaaagaagaagccatcaggactctgcagcgaaaaatttgtgagctgcaagctaggctgcaggcccaggaagaacagcatcaggaagtccagaaggcaaaagaagcagacatagagaagctgaaccaggccttgtgcttgcgctacaagaatgaaaaggagctccaggaagtgatacagcagcagaatgagaagatcctagaacagatagacaagagtggcgagctcataagccttagagaggaggtgacccaccttacccgctcacttcggcgtgcggagacagagaccaaagtgctccaggaggccctggcaggccagctggactccaactgccagcctatggccaccaattggatccaggagaaagtgtggctctctcaggaggtggacaaactgagagtgatgttcctggagatgaaaaatgagaaggaaaaactcatgatcaagttccagagccatagaaatatcctagaggagaaccttcggcgctctgacaaggagttagaaaaactagatgacattgttcagcatatttataagaccctgctctctattccagaggtggtgaggggatgcaaagaactacagggattgctggaatttctgagctaagaaactgaaagccagaatctgcttcacctctttttacctgcaatacccccttaccccaataccaagaccaactggcatagagccaactgagataaatgctatttaaataaagtgtatttaatgaa

SEQ ID NO: 9 - DNA, 5286 bp, Homo sapiens
atcatgtattactggttgccagtgaaggaattaagaggtatggaagtgatccagtcttcaggttttatcatgcctatggcacattaatggaaggtaaaactcaagaagctcttcgagaatttgaggctattaaaaataaacaagatgtatcactttgttctctacttgcactgatatatgcccataaaatgagtcctaatccagatagagaagctattctggaatcagatgccagagtgaaggaacaacgtaaaggagctggagagaaagccttataccatgcaggcttatttttatggcacattggtcgccatgataaagcaagggaatatattgacagaatgatcaaaatatcagatggtagtaaacagggacacgttttgaaagcatggcttgatattacaagaggaaaagagccttacactaaaaaagcactgaagtattttgaagagggactccaagatgggaatgatacttttgctctgctgggtaaggcacaatgccttgagatgcgccagaattattcaggtgccctggagactgtgaaccagataatcgtgaattttccgagcttccttcctgcttttgttaagaaaatgaaattacaactagccttgcaggattgggaccagacagttgagacagcacaaaggttgctgctccaagatagccaaaatgtggaagcactgagaatgcaggcactctactatgtgtgtagagagggggatatagagaaggcttccaccaagctggaaaacttgggaaatacattggatgccatggaaccacagaatgctcaacttttctataacattacactcgccttcagcagaacttgtggacgtagtcaacttattcttcaaaaaattcaaacgttacttgagagagcttttagtttaaaccctcagcaatcagaatttgctacagaacttggataccaaatgattttacaaggaagagttaaagaggcactgaagtggtataagaccgccatgacacttgatgagactagtgtgtctgccctagttggatttatccaatgtcagttgatagaagggcaattacaggatgcagatcagcagctagaatttttaaatgaaatccagcaatccattggaaaatctgcggaattaatctatttacatgcagttcttgccatgaagaaaaataaacgacaagaagaagttattaatttgttaaatgatgtcctggacactcacttttcacaattagaaggtttgcctcttggcatacagtattttgaaaagctaaatcctgatttcttgttagaaattgttatggagtatctgagcttctgtccaatgcagcctgcaagtcctgggcaacctctttgtccacttctcaggcgttgcatctcagtcctggagactgtagtaagaactgttccaggtcttctgcaaacagtcttcctaatagcaaaagtgaaatatttgtcaggtgatattgaagcagctttcaataaccttcagcactgcttagaacacaatccctcttatgctgatgctcatctgctgctagctcaggtttacttgtctcaagaaaaagtcaaattgtgttctcagtctcttgaactttgtctgagctatgattttaaggtgagagactatcctttataccatttgataaaagctcagtcacaaaagaaaatgggagaaatagcagacgcaattaaaacactgcatatggcaatgagtttaccaggaatgaaaagaattggagcttccacaaaatcaaaagacagaaaaactgaagttgatacaagccatcgtttatcgatctttcttgaattgatagacgttcaccgcttaaatggagagcagcatgaggcaaccaaagttttacaagatgccatccatgaattttctggaacatctgaagaagtgcgggttaccattgctaatgcagaccttgctctagcccaaggagatattgaacgggctttaagcatccttcagaatgttacagccgaacagccttattttatagaggccagagaaaaaatggcagatatttatctgaagcacagaaaagataaaatgttatatatcacttgttttagagaaattgctgaaagaatggctaaccctcggtcttttcttctccttggtgatgcatacatgaatattctagagcctgaagaagccatagtagcatatgagcaagcattaaatcagaacccgaaagatggaacattggcaagcaaaatgggcaaagcacttatcaaaactcataactactcaatggcaatcacttactatgaagctgctctgaaaactggacaaaagaattatctttgctatgacctggctgagctcttattaaaattgaaatggtatgacaaagcagaaaaagttcttcagcatgctctggctcatgaacctgtaaatgaactgtcagctctcatggaggatggacgttgtcaagttcttctagcaaaagtttatagtaaaatggaaaaacttggtgatgcgatcactgcattacaacaggctcgagaattacaagctcgggtactaaaacgtgttcagatggaacagccagatgcagttcctgcacagaaacatttagcagctgaaatttgtgcagagattgcaaaacattctgttgctcagcgagactatgaaaaagcaattaagttttatagagaggctctggttcactgcgaaacagataataagattatgttggaactggcacgattatacctggcacaagatgaccctgattcctgcctgcggcagtgtgctctactgcttcagagtgaccaggataacgaagctgctaccatgatgatggctgatctcatgttcagaaaacaagactatgaacaagcagtgtttcatttacagcagcttttagaacgtaagccagataattatatgacattatctcgtttgattgatctcctaagaagatgtggaaaactcgaggatgtcccaagatttttctcaatggctgagaaacgtaactccagagcaaaattggaaccaggatttcagtattgtaaaggactgtatctttggtacactggagaaccaaatgatgcccttcgacattttaataaagctcggaaagatcgtgactggggccaaaatgccctttataatatgatagagatctgtttgaatccagataatgaaactgttggaggtgaagtatttgaaaacctggatggagacctgggtaattcaactgagaagcaagaatctgtgcaactggcagtaagaacagcagaaaaacttcttaaggaactaaaacctcagactgttcagggtcacgtacagcttcgcataatggaaaactattgcttaatggctaccaaacagaaatctaatgttgaacaagcattaaataccttcactgaaatagcagcatctgagaaggagcatatcccagcgctcttgggaatggcaacggcttatatgatcttgaaacagactccacgagccagaaaccagctgaagcgtattgcgaaaatgaattggaatgctattgatgctgaagagtttgagaagagttggctgctacttgctgatatttacattcaatcagcaaaatatgacatggcagaagacctgttaaaacggtgcctgcgtcataatagatcttgctgcaaagcttatgaatatatgggatacattatggaaaaagagcaagcatatacagatgctgccttgaactatgagatggcatggaaatatagcaatcggacaaatccggcagtaggatacaaactggcatttaattacttaaaagcaaaaagatatgtggattcaattgacatatgtcaccaggttcttgaagcacatccaacttatccaaaaatcagaaaggatatacttgataaggcccgtgcgtctttaagaccttgaaaataattttaacttaggtgttggtttaacaggaaatgaaagaaatctaactttcagttcttcctgttcaaaacaggtttgagctcagtgctttgttattagaagtatacccttttttctccagcagaggttgctgctgtacatcaagagaagtactatgtgaaattggtgtttcctaatggagttgaatgagagctggtctatttgactctgttttgattgggtacagatttggtgactctgtggtaaagactataattatttctataaagaatattttgttaaaatctaggtaattaaataccctgtatcttttctaaggaatattatttcaggaaatatatttaaaatgcattgttctcttttaaagtgtttttgttatattcttttatttatttatttatttttaaagacagagccttgatctgccgcccaggctggagtgcagtggcacgatcttggctcactgcaacctccgcctcctgggtttacgcgattctcctgcttcagcctcccgagtagctgggactaaaggcatgtgccatcacacccggctaattttttgtatttttagtagagatgggatttcaccgtgttagccaggaggggcttgatctcttgaccttgtgatccacctgcctcggcctcccaaagtgctgggattacaggcatgagccaccgcacccagcctgtttttgttgtattctgtgttgtttcaaaaattggaataaatctccctgtaaataactcatgaaaaagacaatatatatattttaaatatatattttaataaaggttttataaatagatgatttatattcctcttggaactcaaaagatgtggtaagttttgcaaatcagggtaagctccccctgcattctgtaatgttaatgggtggtggtatagtacagaaaatgtaactttcattgaaaaatcttttttagaaaagggtagagtgtgtgtttccctttcctttcttgagctcattcttcctgctttcaaggccattgtggtcttaagaaataatcaggtcctgaaacctcaatttaaataggtcccttattagggatatttaaccttagcctagaagacttggtctgcaggtataatttcagacactgtaacatttgatggtaaagggtgaccaaatacttttggtcagcagggagtcacaaagcacaccatgtgaaggcaacggtttacccagctctgtttaacagcaccctggcatagaagctttcactctcttacactaaatttaacctaatctaaacttaatccttagcattatttttaatttctcatctacatctttttcaattttccttaaaattgtagtaaacacagtcctcaattttatttgcatttacaataaacagtatttataagtca

SEQ ID NO: 10 - DNA, 5322 bp, Homo sapiens
agtgcggctgcgcgggcgtctcaggctctgaggcccgggcgccgcggctcttttgtttctccgttggggccgagcccgggccctagttggagccggagtcggagtcggagtcggatccggattcggattagcagcccgggaagagtgccgtggcacaggcgccggagggagcgcgaccctcggaccccgcctggcccgcggggctgggacccggccccggcctgcccgatggggcgcgcggccccggagatgcgccctcgcccggccccgcgcccccggccccgcgcccccggcccgcccgccccggcccgcgcctccgcctgagtcccccgcgccttggcccgccaccccccgccccgcgcccccggcccgcctgcgccatggagcccggccgcggcggcacagagaccgtgggcaagttcgagttctcccgcaaggacctgatcggccacggcgccttcgcggtggtcttcaagggccgccaccgcgagaagcacgatttggaggtcgccgtcaagtgcattaacaagaagaacctcgccaagtctcagacgctgctggggaaggaaatcaaaatcctgaaggaactgaaacatgaaaacatcgtggccctgtacgacttccaggaaatggctaattctgtctacctggttatggagtactgcaacggtggggacctggccgactacctgcacgccatgcgcacgctgagcgaggacaccatcaggctcttcctgcagcagatcgcgggcgccatgcggcttctgcacagcaaaggcatcatccaccgcgacctgaaaccgcagaacatcctgctgtccaaccccgccggccgccgcgccaaccccaacagcatccgcgtcaagatcgctgacttcggcttcgcgcggtacctccagagcaacatgatggcggccacactctgcggctcccccatgtacatggcccccgaggtcatcatgtcccagcactacgacgggaaggcggacctgtggagcatcggcaccatcgtctaccagtgcctgacggggaaggcgcccttccaggccagcagcccccaggacctgcgcctgttctacgagaagaacaagacgttggtccccaccatcccccgggagacctcggccccgctgcggcagctgctcctggccctactgcaacgcaaccacaaggaccgcatggacttcgatgagttttttcatcaccctttcctcgatgccagcccctcggtcaggaaatccccacccgtgcctgtgccctcgtacccaagctcggggtccggcagcagctccagcagcagctccacctcccacctggcctccccgccgtccctgggcgagatgcagcagctgcagaagaccctggcctccccggctgacaccgctggcttcctgcacagctcccgggactctggtggcagcaaggactcttcctgtgacacagacgacttcgtcatggtccccgcgcagtttccaggtgacctggtggctgaggcgcccagtgccaaacccccgccagacagcctgatgtgcagtgggagctcactggtggcctctgcgggcttggagagccacggccggaccccatctccatccccaccctgcagcagctcccccagtccctcaggccgggctggcccgttctccagcagcaggtgcggcgcctctgtccccatcccagtccccacgcaggtgcagaactaccagcgcattgagcgaaacctgcagtcacccacccagttccaaacacctcggtcctctgccatccgcaggtcaggcagcaccagccccctgggctttgcaagggccagcccctcgccccctgcccacgctgagcatggaggcgtcctggccaggaagatgtctctgggtggaggccggccctacacgccatctcctcaagttggaaccatccctgagcggccaggctggagcgggacgccctccccacagggagctgagatgcggggtggcaggtcccctcgtccaggctcctctgcacccgagcactctccccgcacttccgggctgggctgccgcctgcacagcgcccccaacctgtctgacttgcacgtcgtccgccccaagctgcccaaaccccccacggaccccctgggagctgtgttcagcccaccacaggccagccctccccagccgtcccacggcctgcagtcctgccggaacctgcggggctcacccaagctgcccgacttcctgcagcgaaaccccctgccccccatcctgggctcccccaccaaggctgtgccctcctttgacttcccgaagacccccagctcccagaacctgctggccctcctagcccggcagggcgtggtgatgacgccccctcgaaaccggacgctgcccgacctctcggaggtgggacccttccatggtcagccgttgggccctggcctgcggccaggcgaggaccccaagggcccctttggccggtctttcagcaccagccgcctcactgacctgctccttaaggcggcgtttgggacacaagccccggacccgggcagcacggagagcctgcaggagaagcccatggagatcgcaccctcagctggctttggagggagcctgcacccaggagcccgtgctgggggcaccagcagcccttccccggtggtcttcaccgtgggctctcccccgagcgggagcacgcccccccagggcccccgcaccaggatgttctcagcgggccccactggctctgccagctcttctgcccgccacctggtgcctgggccctgcagcgaggccccagcccctgagctccctgctccaggacacggctgcagctttgccgaccccattactgcgaacctggagggggctgtgaccttcgaggcccccgacctccctgaggagaccctcatggagcaagagcacacggagatcctgcgtggcctgcgcttcacgctgctgttcgtgcagcacgtcctggagatcgcagccctgaagggcagcgccagtgaggcggcggggggccctgagtaccagctgcaggagagtgtggtggccgaccagatcagcctgctgagccgagaatggggcttcgcggaacagctggtgctgtacctgaaggtggccgagctactgtcctccggcctgcaaagtgccatcgaccagatccgggccggcaagctctgcctgtcgtccactgtgaagcaggtggtgcgcaggctgaatgagctgtacaaggccagcgtggtgtcctgccagggcctgagcctgcggctgcagcgcttcttcctggacaagcagcggctcctggaccgcattcacagcatcactgccgagaggctcatcttcagccacgctgtgcagatggtgcagtcggctgccctggacgagatgttccagcaccgtgagggctgcgtcccacgctaccacaaggccctgctgctcctggaggggctgcagcacatgctctcggaccaggccgacatcgagaacgtcaccaagtgcaagctgtgcattgagcggagactctcggcgctgctgactggcatctgtgcctgacctttctggcctggctgggccccccgtcctgccgagccctgcagagtgggctctgtgtgctggctggactcctcgggacaagcccatggcgctgatcgctggtgctgagccctgccctgggccccacggacagtcagcctgccggcctccctgcagctcacggggcagaaccagcacatctggagccacacagcttggggggtgtctcccatcttttacaggtggggatcacagaatttctgcccctccagctgcctggctcagcaggcgtgggtgccaccaccctctagccccagggcagccccggaggacaggcaagggcctgagaccactgccgactcaaagccaaagcgagctcctgcttagggaaggtcagcaggcactgtgcccaggaagagcctgcggcctcggcgtcccccagtctccaggagcctctccctccgagatacccacccagctttgtcaatcacccaagcactttatgcatatagagacagaacctggacctcaccagggactgctgggcagcgattcctggcagtggcctggtgtttgtacatacacatatgcagacacatgccagggccccccaagcccgagcaccggaccacgttgctgcccaggtctggacctcagcgggagaactggctccggggggagtggggccctgcgctagaggcagaggcagttctttgttcaagcgttcctctggggaccggcagcagaggcaccgtgttctctcagccctggatacgtcttgtaatctttcacactttattcctaaaacgtgtcttatttttatgcagctcattttttctttaaaggagaaaacttgtaggtgtttaagaattggttttgggagggcgaggactgggccaggttagaggcagatggcacaggggcgtgtggcgggcgggtgaggctgctttgcacacctgtgttggtggctgtcccctgccgcccctccctgtggcagcagcaggacaggtgtgtgcccagcaccctccctacctgggcctggaagcagatgaggggaatacttcatgcaaagaaaaaagtaacatgtgcaaaagctccccgtccagctttgacagtcagttttgatgtcagctcctcggcagggtaggcctgatgacagccctgtccctccctgcctctgccttgcccaaggccacggagggcatctgcagagaggcctgccttccggattccaggcgggcatgccctgcaaaccccgcctgggcctcccttggtctgcccagccctcgattagccctgcctgaatcagtagatacttgaacgagtccccagtctgcgggaggcagtggtggggccatggacccatgcggggggttccagggtcacacgccacataacagacaaaaatacacacacgtgtgtttttctttgcaatacttgaaatattgccactgtgcttggacttagaagaagaaaatccccgtgacttcttcctcatcaccttgatggctttattctcaccttgtggggcatgtttgtatttattgcttcatggccgactggaatcctgagtcctgggaagctggcactgcggggatcttgcccggtgtcctggtcctcttgcttccgtcgcggccgcatgtgcgtgtgtccaagcaggtcctgggcgcctcaactgctgcccctggttgaatgttctcttgatagtgctggaccctttgtctattttaaagcgaattttgtgtgatttcctgccctttgcgttatattgtataataccaacgtaaggaaataaacctttggaattgtt

SEQ ID NO: 11 - DNA, 3665 bp, Homo sapiens
tttcaaacagcggaacaaactgaaagctccggtgccagaccccacccccggccccggcccgggaccccctcccctcccgggatcccccggggttcccaccccgcccgcaccgccggggacccggccggtccggcgcgagcccccgtccggggccctggctcggcccccaggttggaggagcccggagcccgccttcggagctacggcctaacggcggcggcgactgcagtctggagggtccacacttgtgattctcaatggagagtgaaaacgcagattcataatgaaaactagcccccgtcggccactgattctcaaaagacggaggctgccccttcctgttcaaaatgccccaagtgaaacatcagaggaggaacctaagagatcccctgcccaacaggagtctaatcaagcagaggcctccaaggaagtggcagagtccaactcttgcaagtttccagctgggatcaagattattaaccaccccaccatgcccaacacgcaagtagtggccatccccaacaatgctaatattcacagcatcatcacagcactgactgccaagggaaaagagagtggcagtagtgggcccaacaaattcatcctcatcagctgtgggggagccccaactcagcctccaggactccggcctcaaacccaaaccagctatgatgccaaaaggacagaagtgaccctggagaccttgggaccaaaacctgcagctagggatgtgaatcttcctagaccacctggagccctttgcgagcagaaacgggagacctgtgcagatggtgaggcagcaggctgcactatcaacaatagcctatccaacatccagtggcttcgaaagatgagttctgatggactgggctcccgcagcatcaagcaagagatggaggaaaaggagaattgtcacctggagcagcgacaggttaaggttgaggagccttcgagaccatcagcgtcctggcagaactctgtgtctgagcggccaccctactcttacatggccatgatacaattcgccatcaacagcactgagaggaagcgcatgactttgaaagacatctatacgtggattgaggaccactttccctactttaagcacattgccaagccaggctggaagaactccatccgccacaacctttccctgcacgacatgtttgtccgggagacgtctgccaatggcaaggtctccttctggaccattcaccccagtgccaaccgctacttgacattggaccaggtgtttaagccactggacccagggtctccacaattgcccgagcacttggaatcacagcagaaacgaccgaatccagagctccgccggaacatgaccatcaaaaccgaactccccctgggcgcacggcggaagatgaagccactgctaccacgggtcagctcatacctggtacctatccagttcccggtgaaccagtcactggtgttgcagccctcggtgaaggtgccattgcccctggcggcttccctcatgagctcagagcttgcccgccatagcaagcgagtccgcattgcccccaaggtttttggggaacaggtggtgtttggttacatgagtaagttctttagtggcgatctgcgagattttggtacacccatcaccagcttgtttaattttatctttctttgtttatcagtgctgctagctgaggaggggatagctcctctttcttctgcaggaccagggaaagaggagaaactcctgtttggagaagggttttctcctttgcttccagttcagactatcaaggaggaagaaatccagcctggggaggaaatgccacacttagcgagacccatcaaagtggagagccctcccttggaagagtggccctccccggccccatctttcaaagaggaatcatctcactcctgggaggattcgtcccaatctcccaccccaagacccaagaagtcctacagtgggcttaggtccccaacccggtgtgtctcggaaatgcttgtgattcaacacagggagaggagggagaggagccggtctcggaggaaacagcatctactgcctccctgtgtggatgagccggagctgctcttctcagaggggcccagtacttcccgctgggccgcagagctcccgttcccagcagactcctctgaccctgcctcccagctcagctactcccaggaagtgggaggaccttttaagacacccattaaggaaacgctgcccatctcctccaccccgagcaaatctgtcctccccagaacccctgaatcctggaggctcacgcccccagccaaagtagggggactggatttcagcccagtacaaacctcccagggtgcctctgaccccttgcctgaccccctggggctgatggatctcagcaccactcccttgcaaagtgctcccccccttgaatcaccgcaaaggctcctcagttcagaacccttagacctcatctccgtcccctttggcaactcttctccctcagatatagacgtccccaagccaggctccccggagccacaggtttctggccttgcagccaatcgttctctgacagaaggcctggtcctggacacaatgaatgacagcctcagcaagatcctgctggacatcagctttcctggcctggacgaggacccactgggccctgacaacatcaactggtcccagtttattcctgagctacagtagagccctgcccttgcccctgtgctcaagctgtccaccatcccgggcactccaaggctcagtgcaccccaagcctctgagtgaggacagcaggcagggactgttctgctcctcatagctccctgctgcctgattatgcaaaagtagcagtcacaccctagccactgctgggaccttgtgttccccaagagtatctgattcctctgctgtccctgccaggagctgaagggtgggaacaacaaaggcaatggtgaaaagagattaggaaccccccagcctgtttccattctctgcccagcagtctcttaccttccctgatctttgcagggtggtccgtgtaaatagtataaattctccaaattatcctctaattataaatgtaagcttatttccttagatcattatccagagactgccagaaggtgggtaggatgacctggggtttcaattgacttctgttccttgcttttagttttgatagaagggaagacctgcagtgcacggtttcttccaggctgaggtacctggatcttgggttcttcactgcagggacccagacaagtggatctgcttgccagagtcctttttgcccctccctgccacctccccgtgtttccaagtcagctttcctgcaagaagaaatcctggttaaaaaagtcttttgtattgggtcaggagttgaatttggggtgggaggatggatgcaactgaagcagagtgtgggtgcccagatgtgcgctattagatgtttctctgataatgtccccaatcataccagggagactggcattgacgagaactcaggtggaggcttgagaaggccgaaagggcccctgacctgcctggcttccttagcttgcccctcagctttgcaaagagccaccctaggccccagctgaccgcatgggtgtgagccagcttgagaacactaactactcaataaaagcgaaggtggacatgaaaaaaaaaaaaaaaaaaa

SEQ ID NO: 12 - DNA, 2375 bp, Homo sapiens
aggctgctcccggacaagggcaacgagcgtttcgtttggacttctcgacttgagtgcccgcctccttcgccgccgcctctgcagtcctcagcgcagttatgcccagttcttcccgctgtggggacacgaccacggaggaatccttgcttcagggactcgggaccctgctggaccccttcctcgggtttaggggatgtggggaccaggagaaagtcaggatccctaagagtcttccctgcctggatggatgagtggcttcttctccacctagattctttccacaggagccagcatacttcctgaacatggagagtgttgttcgccgctgcccattcttatcccgagtcccccaggcctttctgcagaaagcaggcaaatctctgttgttctatgcccaaaactgccccaagatgatggaagttggggccaagccagcccctcgggcattgtccactgcagcagtacactaccaacagatcaaagaaacccctccggccagtgagaaagacaaaactgctaaggccaaggtccaacagactcctgatggatcccagcagagtccagatggcacacagcttccgtctggacaccccttgcctgccacaagccagggcactgcaagcaaatgccctttcctggcagcacagatgaatcagagaggcagcagtgtcttctgcaaagccagtcttgagcttcaggaggatgtgcaggaaatgaatgccgtgaggaaagaggttgctgaaacctcagcaggccccagtgtggttagtgtgaaaaccgatggaggggatcccagtggactgctgaagaacttccaggacatcatgcaaaagcaaagaccagaaagagtgtctcatcttcttcaagataacttgccaaaatctgtttccacttttcagtatgatcgtttctttgagaaaaaaattgatgagaaaaagaatgaccacacctatcgagtttttaaaactgtgaaccggcgagcacacatcttccccatggcagatgactattcagactccctcatcaccaaaaagcaagtgtcagtctggtgcagtaatgactacctaggaatgagtcgccacccacgggtgtgtggggcagttatggacactttgaaacaacatggtgctggggcaggtggtactagaaatatttctggaactagtaaattccatgtggacttagagcgggagctggcagacctccatgggaaagatgccgcactcttgttttcctcgtgctttgtggccaatgactcaaccctcttcaccctggctaagatgatgccaggctgtgagatttactctgattctgggaaccatgcctccatgatccaagggattcgaaacagccgagtgccaaagtacatcttccgccacaatgatgtcagccacctcagagaactgctgcaaagatctgacccctcagtccccaagattgtggcatttgaaactgtccattcaatggatggggcggtgtgcccactggaagagctgtgtgatgtggcccatgagtttggagcaatcaccttcgtggatgaggtccacgcagtggggctttatggggctcgaggcggagggattggggatcgggatggagtcatgccaaaaatggacatcatttctggaacacttggcaaagcctttggttgtgttggagggtacatcgccagcacgagttctctgattgacaccgtacggtcctatgctgctggcttcatcttcaccacctctctgccacccatgctgctggctggagccctggagtctgtgcggatcctgaagagcgctgagggacgggtgcttcgccgccagcaccagcgcaacgtcaaactcatgagacagatgctaatggatgccggcctccctgttgtccactgccccagccacatcatccctgtgcgggttgcagatgctgctaaaaacacagaagtctgtgatgaactaatgagcagacataacatctacgtgcaagcaatcaattaccctacggtgccccggggagaagagctcctacggattgcccccacccctcaccacacaccccagatgatgaactacttccttgagaatctgctagtcacatggaagcaagtggggctggaactgaagcctcattcctcagctgagtgcaacttctgcaggaggccactgcattttgaagtgatgagtgaaagagagaagtcctatttctcaggcttgagcaagttggtatctgctcaggcctgagcatgacctcaattatttcacttaaccccaggccattatcatatccagatggtcttcagagttgtctttatatgtgaattaagttatattaaattttaatctatagtaaaaacatagtcctggaaataaattcttgcttaaatggtg

SEQ ID NO: 13 - DNA, 1392 bp, Homo sapiens
cctttgcctgctcaccgccagcgtaggtgctaccaccgctgccgtcgccgccgccattttgatggcaggaagagtccggttctgggacagctggagacagtggtggtgactgaaataactttaccaaaggaaagctattttgcgaactatcttctccagcggagatggccaatgtgctttgtaacagagccagactggtttcctatctcccaggattttgctctttagttaaaagggttgtcaatcccaaagccttttcgactgcaggatcatcaggttcggatgagtctcatgtggctgctgcacctccagatatatgctctcgaacagtgtggcctgatgaaactatgggaccctttggacctcaagatcagaggttccagcttcctgggaacataggttttgattgtcacctcaatgggactgcttcacagaagaaaagcctggttcataaaactttgcctgatgttctagcagaacctttatcaagtgaaagacatgagtttgtgatggcacaatatgtgaatgaatttcagggtaatgatgcacctgttgaacaagaaattaacagtgcagaaacttactttgaaagtgccagagtagagtgtgcaatacagacatgtccagaattgctgcgaaaagattttgaatcactgtttccagaagtagctaatggcaaactaatgattctgactgtaacacaaaaaactaagaatgatatgactgtttggagtgaagaagtagaaattgaaagagaagtgctcttagaaaagttcatcaatggtgctaaggaaatttgctatgctcttcgagctgagggttattgggctgactttattgacccatcatctggtttggcattttttggaccatatacaaacaacactctttttgaaactgatgaacgctaccgacatttaggattctctgttgatgaccttggatgctgtaaagtgattcgtcatagtctctggggtacccatgtagttgtagggagtatcttcactaatgcaacaccagacagccatattatgaagaaattaagtggaaattagcagaaatatccattcatttgctgtactatttgtatgtaatatttgggttgatctataaacactgtcagactaaagtttttaaaatatatttatttctaagtatttatttcagcatttatgaatttacaacattggcaagtgatttgggattttaaaattgcaaatgttcatttattcatatcattgaatacacgttgaacacatccacattgtataggatgtggtaattagcttgtaaccagggtatgatctgctattgttatttctcctctttattggaaaaaggcctcagttttaattattttcttcccaaaataaatcacacatttggttacaa

SEQ ID NO: 14 - DNA, 4582 bp, Homo sapiens
acagagagccgagctctggagcctcagcgagcggaggaggaggcgcagcggccgacggccgagtactgcggtgagagccagcgggccagcgccagcctcaacagccgccagaagtacacgaggaaccggcggcggcgtgtgcgtgtaggcccgtgtgcgggcggcggcgcgggagcagcgcggagcggcagccggctggggcgggtggcatcatggacgagaaggtgttcaccaaggagctggaccagtggatcgagcagctgaacgagtgcaagcagctgtccgagtcccaggtcaagagcctctgcgagaaggctaaagaaatcctgacaaaagaatccaacgtgcaagaggttcgatgtccagttactgtctgtggagatgtgcatgggcaatttcatgatctcatggaactgtttagaattggtggcaaatcaccagatacaaattacttgtttatgggagattatgttgacagaggatattattcagttgaaacagttacactgcttgtagctcttaaggttcgttaccgtgaacgcatcaccattcttcgagggaatcatgagagcagacagatcacacaagtttatggtttctatgatgaatgtttaagaaaatatggaaatgcaaatgtttggaaatattttacagatctttttgactatcttcctctcactgccttggtggatgggcagatcttctgtctacatggtggtctctcgccatctatagatacactggatcatatcagagcacttgatcgcctacaagaagttccccatgagggtccaatgtgtgacttgctgtggtcagatccagatgaccgtggtggttggggtatatctcctcgaggagctggttacacctttgggcaagatatttctgagacatttaatcatgccaatggcctcacgttggtgtctagagctcaccagctagtgatggagggatataactggtgccatgaccggaatgtagtaacgattttcagtgctccaaactattgttatcgttgtggtaaccaagctgcaatcatggaacttgacgatactctaaaatactctttcttgcagtttgacccagcacctcgtagaggcgagccacatgttactcgtcgtaccccagactacttcctgtaatgaaattttaaacttgtacagtattgccatgaaccatatatcgacctaatggaaatgggaagagcaacagtaactccaaagtgtcagaaaatagttaacattcaaaaaacttgttttcacatggaccaaaagatgtgccatataaaaatacaaagcctcttgtcatcaacagccgtgaccactttagaatgaaccagttcattgcatgctgaagcgacattgttggtcaagaaaccagtttctggcatagcgctatttgtagttacttttgctttctctgagagactgcagataataagatgtaaacattaacacctcgtgaatacaatttaacttccatttagctatagctttactcagcatgactgtagataaggatagcagcaaacaatcattggagcttaatgaacatttttaaaaataattaccaaggcctcccttctacttgtgagttttgaaattgttctttttattttcagggataccgtttaatttaattatatgatttgtctgcactcagtttattccctactcaaatctcagccccatgttgttctttgttattgtcagaacctggtgagttgttttgaacagaactgttttttccccttcctgtaagacgatgtgactgcacaagagcactgcagtgtttttcataataaacttgtgaactaagaactgagaaggtcaaattttaattgtatcaatgggcaagactggtgctgtttattaaaaaagttaaatcaattgagtaaattttagaatttgtagacttgtaggtaaaataaaaatcaagggcactacataacctctctggtaactccttgacattcttcagattaacttcaggatttatttgtatttcacatattacaatttgtcacattgttggtgtgcactttgtgggttcttcctgcatattaacttgtttgtaagaaaggaaatctgtgctgcttcagtaagacttaattgtaaaaccatataacttgagatttaagtctttgggttttgttttaataaaacagcatgttttcaggtagagcttaaactaaatgatgtgtttacttagtgcagtttctggttatgaatattatattgctatgtgtatattatatggactctttaaaatgattgacagattggcaaattcttaaatctttgtacattgttgagtcatatgttcttagagttaaatttgtctcagataagaaagtgttaaagcattagcctgtgtcaagttctttgagtgatactagtgaaaccaaatagaaaactattgttggatcatgatttagtcttatgtacattcacccgaagacaaaaatggtacttaaagtggcagtgttcaacatttaatgagtttttccccttttatccttcgaataggattagatgtttaaaaaaaagttcttctgtgggaactaatatttgatattttaacctaccagagtaaacaggaacacttaatcatacttgtgagtgtagtaaataaaagttttcttgctttgtgctgtgttgaatctggaaccaacagggaagttatagcatatcccctttctaaaatgcttgaggaacacatacataccgaatgtcttttctgatctaattgatagtatttttagtggcttgtggagttaattttccaaagcaaaaggccattagggtttctacatttcatttcatttcattcttttctttcacaagaaatacattctctgtgtgtctttttgttgctctgtcactctatgccctttctctccgactgaacaaatagcttatccatgtgcagtggttttaatacccaaacaatctagacaccaagcagctattttttccggtcctgtgatatcagaattgaccaaggaatacgtatattgtaattgacacgtggtggtatcttccaggtacaaattctctaaattttgtggttagcagaatgggacttgtgataagaatagcttggttttagcataactagggtttaaaataattgtttaattatagagactgaccgggctttggccatctaaactggaaagtgttagtaccctaccttcttttgaaaatggctatggtaaggaaaatgtgttagtaaattatgtattttcttgaaaaatacataattatggttggatgggaatcactaagttgggtgttaactgatgtctcaattagtaacattaggattttcattaataaacctaaaaagctttccctaagaacaggcctggcacagtggctcatgcctgtaatcccagcactttgggagaccagggtgggtggatcccttgaggtcaggagttgaagagcagcctggccaacatggcaaaaccccatctctacaaaaaatatgaaaatcagccgggcttggtggcataccatagtcccagctacttgggaggctgaggtgagaggatcgcctgagcccaggagatggaggttgcagtgggctgagattgtgccactgtactccagtctgggtgacagagccagaccctgtctcaaaaataaagaggattctgagtttgtatagtgagggcttgcagaaattttgaaacttattttgtaagtttacaatgaatttgtacatgatgtgctcatgtcttgggttgagtatcctagacatgattttttcatttgctgcatattaaacatttgttggttgtagtcggtatttcttaaatagaagtttgtcaatattagattagtttcaagaaggacttagctcaggaaaaggatagttatttctgtggttctcagctttgatgcctacagagattctgatttaaattgctggaggagggcccaggcatacattttttaagtttcccaagtgattctaatttacatctagggttaaaaacagccaggcgcggtggctcatgcctgtaatcccagcacttggggaggccggggtgggtggatcacctgatgtcaggagatcgagaccagcctggccagcgtggtgaaaccccatctctattaaaaatacaaaactgaccggtgtggtggcaggagcctgtaatcccagctacttgggaggctgaggcaggagaatcacttgaactcaggaggaggaggttacagtgagcccagatcgtgccattgcactccagcctgggcaaaaagagcaaaactccatctcaaaaaacaaaaacacctcactgctgtttcctaagtacatacttaagaaaattgggatacatggtggtggttcatggatgttgataaggaattaaaatgtaccgtgcgactctctgtttcagtggtgacttttacctgtttagtataaatattcctttgcttccaaccataaatgtgttcttagaaatgggcctatagtttagtaacctatagtttggtaataggcttgtttgttttcagatggattttggttctgtgagctaaagctattttgcattaaagccttcgtcctcaca

SEQ ID NO: 15 - DNA, 5234 bp, Homo sapiens
agagcgtcgggatatcgggtggcggctcgggacggaggacgcgctagtgtgagtgcgggcttctagaactacaccgaccctcgtgtcctcccttcatcctgcggggctggctggagcggccgctccggtgctgtccagcagccatagggagccgcacggggagcgggaaagcggtcgcggccccaggcggggcggccgggatggagcggggccgcgagcctgtggggaaggggctgtggcggcgcctcgagcggctgcaggttcttctgtgtggcagttcagaatgatggatcaagctagatcagcattctctaacttgtttggtggagaaccattgtcatatacccggttcagcctggctcggcaagtagatggcgataacagtcatgtggagatgaaacttgctgtagatgaagaagaaaatgctgacaataacacaaaggccaatgtcacaaaaccaaaaaggtgtagtggaagtatctgctatgggactattgctgtgatcgtctttttcttgattggatttatgattggctacttgggctattgtaaaggggtagaaccaaaaactgagtgtgagagactggcaggaaccgagtctccagtgagggaggagccaggagaggacttccctgcagcacgtcgcttatattgggatgacctgaagagaaagttgtcggagaaactggacagcacagacttcaccggcaccatcaagctgctgaatgaaaattcatatgtccctcgtgaggctggatctcaaaaagatgaaaatcttgcgttgtatgttgaaaatcaatttcgtgaatttaaactcagcaaagtctggcgtgatcaacattttgttaagattcaggtcaaagacagcgctcaaaactcggtgatcatagttgataagaacggtagacttgtttacctggtggagaatcctgggggttatgtggcgtatagtaaggctgcaacagttactggtaaactggtccatgctaattttggtactaaaaaagattttgaggatttatacactcctgtgaatggatctatagtgattgtcagagcagggaaaatcacctttgcagaaaaggttgcaaatgctgaaagcttaaatgcaattggtgtgttgatatacatggaccagactaaatttcccattgttaacgcagaactttcattctttggacatgctcatctggggacaggtgacccttacacacctggattcccttccttcaatcacactcagtttccaccatctcggtcatcaggattgcctaatatacctgtccagacaatctccagagctgctgcagaaaagctgtttgggaatatggaaggagactgtccctctgactggaaaacagactctacatgtaggatggtaacctcagaaagcaagaatgtgaagctcactgtgagcaatgtgctgaaagagataaaaattcttaacatctttggagttattaaaggctttgtagaaccagatcactatgttgtagttggggcccagagagatgcatggggccctggagctgcaaaatccggtgtaggcacagctctcctattgaaacttgcccagatgttctcagatatggtcttaaaagatgggtttcagcccagcagaagcattatctttgccagttggagtgctggagactttggatcggttggtgccactgaatggctagagggatacctttcgtccctgcatttaaaggctttcacttatattaatctggataaagcggttcttggtaccagcaacttcaaggtttctgccagcccactgttgtatacgcttattgagaaaacaatgcaaaatgtgaagcatccggttactgggcaatttctatatcaggacagcaactgggccagcaaagttgagaaactcactttagacaatgctgctttccctttccttgcatattctggaatcccagcagtttctttctgtttttgcgaggacacagattatccttatttgggtaccaccatggacacctataaggaactgattgagaggattcctgagttgaacaaagtggcacgagcagctgcagaggtcgctggtcagttcgtgattaaactaacccatgatgttgaattgaacctggactatgagaggtacaacagccaactgctttcatttgtgagggatctgaaccaatacagagcagacataaaggaaatgggcctgagtttacagtggctgtattctgctcgtggagacttcttccgtgctacttccagactaacaacagatttcgggaatgctgagaaaacagacagatttgtcatgaagaaactcaatgatcgtgtcatgagagtggagtatcacttcctctctccctacgtatctccaaaagagtctcctttccgacatgtcttctggggctccggctctcacacgctgccagctttactggagaacttgaaactgcgtaaacaaaataacggtgcttttaatgaaacgctgttcagaaaccagttggctctagctacttggactattcagggagctgcaaatgccctctctggtgacgtttgggacattgacaatgagttttaaatgtgatacccatagcttccatgagaacagcagggtagtctggtttctagacttgtgctgatcgtgctaaattttcagtagggctacaaaacctgatgttaaaattccatcccatcatcttggtactactagatgtctttaggcagcagcttttaatacagggtagataacctgtacttcaagttaaagtgaataaccacttaaaaaatgtccatgatggaatattcccctatctctagaattttaagtgctttgtaatgggaactgcctctttcctgttgttgttaatgaaaatgtcagaaaccagttatgtgaatgatctctctgaatcctaagggctggtctctgctgaaggttgtaagtggtcgcttactttgagtgatcctccaacttcatttgatgctaaataggagataccaggttgaaagaccttctccaaatgagatctaagcctttccataaggaatgtagctggtttcctcattcctgaaagaaacagttaactttcagaagagatgggcttgttttcttgccaatgaggtctgaaatggaggtccttctgctggataaaatgaggttcaactgttgattgcaggaataaggccttaatatgttaacctcagtgtcatttatgaaaagaggggaccagaagccaaagacttagtatattttcttttcctctgtcccttcccccataagcctccatttagttctttgttatttttgtttcttccaaagcacattgaaagagaaccagtttcaggtgtttagttgcagactcagtttgtcagactttaaagaataatatgctgccaaattttggccaaagtgttaatcttaggggagagctttctgtccttttggcactgagatatttattgtttatttatcagtgacagagttcactataaatggtgtttttttaatagaatataattatcggaagcagtgccttccataattatgacagttatactgtcggttttttttaaataaaagcagcatctgctaataaaacccaacagatactggaagttttgcatttatggtcaacacttaagggttttagaaaacagccgtcagccaaatgtaattgaataaagttgaagctaagatttagagatgaattaaatttaattaggggttgctaagaagcgagcactgaccagataagaatgctggttttcctaaatgcagtgaattgtgaccaagttataaatcaatgtcacttaaaggctgtggtagtactcctgcaaaattttatagctcagtttatccaaggtgtaactctaattcccattttgcaaaatttccagtacctttgtcacaatcctaacacattatcgggagcagtgtcttccataatgtataaagaacaaggtagtttttacctaccacagtgtctgtatcggagacagtgatctccatatgttacactaagggtgtaagtaattatcgggaacagtgtttcccataattttcttcatgcaatgacatcttcaaagcttgaagatcgttagtatctaacatgtatcccaactcctataattccctatcttttagttttagttgcagaaacattttgtggtcattaagcattgggtgggtaaattcaaccactgtaaaatgaaattactacaaaatttgaaatttagcttgggtttttgttacctttatggtttctccaggtcctctacttaatgagatagtagcatacatttataatgtttgctattgacaagtcattttaactttatcacattatttgcatgttacctcctataaacttagtgcggacaagttttaatccagaattgaccttttgacttaaagcagagggactttgtatagaaggtttgggggctgtggggaaggagagtcccctgaaggtctgacacgtctgcctacccattcgtggtgatcaattaaatgtaggtatgaataagttcgaagctccgtgagtgaaccatcattataaacgtgatgatcagctgtttgtcatagggcagttggaaacggcctcctagggaaaagttcatagggtctcttcaggttcttagtgtcacttacctagatttacagcctcacttgaatgtgtcactactcacagtctctttaatcttcagttttatctttaatctcctcttttatcttggactgacatttagcgtagctaagtgaaaaggtcatagctgagattcctggttcgggtgttacgcacacgtacttaaatgaaagcatgtggcatgttcatcgtataacacaatatgaatacagggcatgcattttgcagcagtgagtctcttcagaaaacccttttctacagttagggttgagttacttcctatcaagccagtacgtgctaacaggctcaatattcctgaatgaaatatcagactagtgacaagctcctggtcttgagatgtcttctcgttaaggagatgggccttttggaggtaaaggataaaatgaatgagttctgtcatgattcactattctagaacttgcatgacctttactgtgttagctctttgaatgttcttgaaattttagactttctttgtaaacaaatgatatgtccttatcattgtataaaagctgttatgtgcaacagtgtggagattccttgtctgatttaataaaatacttaaacactgaaaaaaaaaaa

SEQ ID NO: 16 - DNA, 8369 bp, Homo sapiens
agccgtttccggagtctgcgctgcgcccggttccgccattgcggctctcctggcccctggagcctccgcccccgacccgagctctttcgtctgcctgccagtttcctgcgtccccggagaggatcctgctgagcccagcctcccccctccccttctcctcctctcccttggagagcccgggcagccactgccccgcagccccagtgacaggaggagaccataacccccgacagcgccatggcccagattctgccaattcgttttcaggagcatctccagctccagaacctgggtatcaacccagcaaacattggcttcagtaccctgactatggagtctgacaaattcatctgcattagagaaaaagtaggagagcaggcccaggtggtaatcattgatatgaatgacccaagtaatccaattcgaagaccaatttcagcagacagcgccatcatgaatccagctagcaaagtaattgcactgaaagctgggaaaactcttcagatttttaacattgaaatgaaaagtaaaatgaaggctcataccatgactgatgatgtcaccttttggaaatggatctctttgaatacggttgctcttgttacggataatgcagtttatcactggagtatggaaggagagtctcagccagtgaaaatgtttgatcgccattctagccttgcagggtgccagattatcaattaccgtacagatgcaaaacaaaagtggttacttctgactggtatatctgcacagcaaaatcgtgtggtgggagctatgcagctatattctgtagataggaaagtgtctcagcccattgaaggacatgcagctagctttgcacagtttaagatggaaggaaatgcagaagaatcaacgttattttgttttgcagttcggggccaagctggagggaagttacatattattgaagttggcacaccacctacagggaaccagccctttccaaagaaggcagtggatgtcttctttcctccagaagcacaaaatgattttcctgttgcaatgcagatcagtgaaaagcatgatgtggtgttcttgataaccaagtatggttatatccacctctatgatcttgagactggtacctgcatctacatgaatagaatcagtggagaaacaatttttgttactgcacctcatgaagccacagctggaataattggagtaaacagaaagggacaagttctgtcagtgtgtgtggaagaagaaaacataattccttacatcaccaatgttctacaaaatcctgatttggctctgagaatggctgtacgtaataacttagccggtgctgaagaactctttgcccggaaatttaatgctctttttgcccagggaaattactcggaggcagcaaaggtggctgctaatgcaccaaagggaattcttcgtactccagacactatccgtcggttccagagtgtcccagcccagccaggtcaaacttctcctctacttcagtactttggtatccttttggaccagggacagctcaacaaatacgaatccttagagctttgtaggcctgtacttcagcaagggcgaaaacagcttttggagaaatggttaaaagaagataagctggaatgttctgaagaactgggtgatcttgtgaaatctgtggaccctacattggcacttagtgtgtacctaagggctaacgtcccaaataaagtcattcagtgctttgcagaaacaggtcaagtccaaaagattgttttatatgctaaaaaagttggatacactccagattggatatttctgctgagaaatgtaatgcgaatcagtccagatcagggacagcagtttgcccaaatgttagttcaagatgaagagcctcttgctgacatcacacagattgtagatgtctttatggaatacaatctaattcagcagtgtactgcattcttgcttgatgctctgaagaataatcgcccatctgaaggtcctttacagacgcggttacttgagatgaaccttatgcatgcgcctcaagttgcagatgctattctaggcaatcagatgttcacacattatgaccgggctcatattgctcaactgtgtgaaaaggctggcctactgcagcgtgcattagaacatttcactgatttatatgatataaaacgtgcagtggttcacacccatcttcttaaccctgagtggttagtcaactactttggttccttatcagtagaagactccctagaatgtctcagagccatgctgtctgccaacatccgtcagaatctgcagatttgtgttcaggtggcttctaaatatcatgaacaactgtcaactcagtctctgattgaactttttgaatctttcaagagttttgaaggtctcttttattttctgggatccattgttaactttagccaggacccagatgtgcactttaaatatattcaggcagcttgcaagactgggcaaatcaaagaagtagaaagaatctgtagagaaagcaactgctacgatcctgagcgagtcaagaattttcttaaggaagcaaaactaacagatcagctaccacttatcattgtgtgtgatcgatttgactttgtccatgatttggtgctctatttatatagaaataatcttcaaaagtatatagagatatatgtacagaaggtgaatccaagtcgacttcctgtagttattggaggattacttgatgttgactgttctgaagatgtcataaaaaacttgattcttgttgtaagaggtcaattctctactgatgagcttgttgctgaggttgaaaaaagaaacagattgaaactgcttctgccttggctagaggccagaattcatgagggctgtgaggagcctgctactcacaatgccttagccaaaatctacatagacagtaataacaacccggagagatttcttcgtgaaaatccctactatgacagtcgcgttgttggaaagtattgtgagaagagagatccacatctggcctgtgttgcttatgaacgtggccaatgtgatctggaacttattaatgtttgcaatgagaattccctcttcaaaagtctttctcgctacctggtacgtcgaaaggatccagaattgtggggcagcgtgctgctggaaagcaatccttacaggagacccctaattgaccaggttgtacaaacagctttgtctgagactcaggaccctgaagaagtgtcagtaactgtaaaggctttcatgactgcagaccttcctaatgaactcattgaactgctggagaaaattgtccttgataactctgtattcagtgaacacaggaatctgcaaaacctccttatcctcactgcaattaaggctgaccgtacacgtgttatggagtatattaaccgcctggataattatgatgccccagatattgccaatatcgccatcagcaatgagctgtttgaagaagcatttgccattttccggaaatttgatgtcaatacttcagcagttcaggtcttaattgagcatattggaaacttggatcgggcatatgagtttgctgaacgttgcaatgaacctgcggtctggagtcaacttgcaaaagcccagttgcagaaaggaatggtgaaagaagccattgattcttatatcaaagcagatgatccttcctcctacatggaagttgttcaggctgccaatactagtggaaactgggaagaactggtgaagtacttgcagatggcccgtaagaaggctcgagagtcctatgtggagacagaactgatattcgcactggctaaaacaaaccgccttgcagagttagaagaatttatcaatggaccaaataatgctcatatccaacaagttggtgaccgttgttatgatgaaaaaatgtatgatgctgctaagttgttgtacaataatgtttccaattttggacgtttggcatctaccctggttcacctgggtgaatatcaggcagctgttgatggggctaggaaagctaacagtactcgaacatggaaagaggtctgcttcgcctgtgtagatgggaaagaattccgtcttgctcagatgtgtggacttcatattgttgtacatgcagatgaattagaagaacttatcaactactatcaggatcgtggctattttgaagagctgatcaccatgttggaagcagcactgggacttgagcgagctcacatgggaatgtttactgaattagctattctatactctaaatttaagcctcagaaaatgagggagcacctggagctgttctggtctagagtgaatattcccaaggtgctaagagctgcagaacaagctcatctttgggcagaactggtgtttttgtatgacaagtatgaagaatatgataatgccataattaccatgatgaatcatccaactgatgcctggaaagaagggcaattcaaagatatcattaccaaggttgccaatgtggaactatactacagagcaatacagttctacttagaattcaagcctctgttgttaaatgatttgctgatggtgctgtctccacggttggatcacactcgtgcagtcaattatttcagcaaggttaaacagctaccactggtgaaaccgtatttgcgttcagttcagaaccataacaacaaatctgtgaatgaatcattgaacaatctttttattacagaagaagattatcaggctctgcgaacatcaatagatgcttatgacaactttgacaatatctcgcttgctcagcgtttggaaaaacatgaactcattgagttcaggagaattgctgcttatctcttcaaaggcaacaatcgctggaaacagagtgtagagctgtgcaagaaagacagcctttacaaggatgcaatgcagtatgcttctgaatctaaagatactgaattggctgaagaactcctgcagtggtttttgcaggaagaaaaaagagagtgctttggagcttgtctgtttacctgttacgatcttttaaggccagatgtcgtcctagaaactgcatggaggcacaatatcatggattttgccatgccctatttcatccaggtcatgaaggagtacttgacaaaggtggataaattagatgcttcagaatcactgagaaaagaagaagaacaagctacagagacacaacccattgtttatggtcagccccagttgatgctgacagcaggacccagtgttgccgtccctccccaggcaccttttggttatggttataccgcaccaccgtatggacagccacagcctggctttgggtacagcatgtgagatgaagcgctgatcctgtagtcacctattttcgtactgaaacatcgtctttacccacttctcagtttataatgggggaaaacaggcaacgtgttcttgtaacctttatttcatgaaggacttctttttgtttctaactataaacttggatcacctatgttaaaaccttatttcacattccacatcattttagaatttattttcgaaggggaatagtttcaatgttttattcacttgggctttttttcttccccctctttctttaaagaactgctcaatattcaatctgttgtgaagaacctgatttgcactctgtagtgtttaaagaaacaaagaaactctaatattgaatctcttaaatttagtgtatgtaaacagcttacaaatacgtattgtctaaatgcatttaaatctgttttattcaaagaaaagctaaagcaaaaacactggcatatgaccatgcaagactgtcagtgccaacaaagacaacactaatcagcacatcgtacactggattgcagtgcttcccagattattgaaaaatgttacagacaacttgcctgatttttaaatgagcgtaaaaggccctctaacctatgcaggtttccccattatgcatatagaaaatgctagtatgttttgctcacttcatatgtaacaggtgcccttatgttgtgctgtatcctgtgctttttctgtgggaccattccattcaggagcaaagagcaccatgattccaatcttgtgtgtgtttactaacccttccctgaggtttgtgtatgttggatattgtggtgttttagatcactgagtgtacagaagagagaaattcaaacaaaatattgctgttcttcagttttgtttgtggaatttgaaattactcaaatttaaaataaattactggactgtggaaataacatagaattgaagttttaattaaataccactcaaacgaaaagaacagtagtttttgtagttttatattggatactgaggcattagggaggcatgaaaggaagaggaatgaggattgagacatgtgaagacattgtgcattatatcaatgtgcattcctgtagttcattaacaaggtacatgcaatagtctaaagaaccagagtcactactatagtggcttaacatttaatctgtctccaatattttaaccaagtgacaccgaggtttttatcgaagcatttcacttaaatgaacaaatcatggctgttatattaacttgaaataaaatatatttaaacatgtagttaacatgctctttctcatcatgaattataaaggtgcccaaattatgggtatcttgatttttttcaaaaattggttgtgtgaatccagctcttgcttatggctgagaatgttcctaaagttcatttcactatcccttaatcctcaatagctacacatacccccttgcctagttagtcttgcactgctttacaactctcttaggcaaattacctaacataagctccacagaagagttttttaaaacttaaaatccctgtcccaccaggtgtggtggctcatgcctgtaatcccagcactttgggaggctgaggcaggcggattgcttgaggccaggagttcgagacaagcctgaccaacatggtgactccatctctactaaaaataaaaaatcagccaggtgtgatggtggatgcctataagatcctagctgctactcaggaggcaggaggctgaggcatgagaatcacttgaacctgtgaggcaaaggttgtagtgagccaagatcacgtcactgcactccatcctgggtgacagaatgagactcttgtctcaaaaaacaaaaaaacctatttagtttcatccaggacattaagtgaaagtgtttaatgtgagtgcaggtcagtgaagaatacaatggtgcccctgctttgatttgtgggaggtgccatcagttttccccaccactgcttttgcaccctcagtgcaaatatcaacacagagaaaaaaaaaataataatagtattatgaaaacattgactctgtggagaccctgtgggttctgcagagtatactttgaaaactataagattatgagttctataaaataccaagtacagatgaactagaaaacaagcatatatccacaattaccagaattttcatagtattccttttagtagatatgccatgacagttacttagccaccccatgccatcctgttgggaatgccactacctttgaatttggagccatcagtctatctgaggcaaacctcagaaattacctgagccagaatcatgcacttagcactgagttcaactcagtcttaacgttgcattttgttgcatcacttttgcagccagtaaacattctgtttagaaatagttgctattgtggcatcattcacagttgcaatttttctcctgtgctgtcatatgcctgtgcgaagtgtattaaatgaatcaaatattagaaatttcaaggctgtctttagtgttctgcccacaatactccaccaatgaccttagaccttgagatggtgctataacgctgcttatattgcagttaaccatagagaggtggagccacttaaaatgggcctattaccaaaattctccctggcatcattacagttcttggggatacactgattttagaaattactgtcagtatcctcctaaaagaaggcttaaatagtttctaacaagatgactatcaggaagctatgtggcttggggagttgggaccctctgcctcatattctgggtaactggtataacatagtaattattaggattgtatcaagtgtatctaaagatcaaaagggaaaaaaggcacccttaattgtcaaagttagttctaggaaaaaatactagcagggatgacaaactacgttcactttacagttaccataaattcttacttgggcccacccatttccatctgttaaggtccataaggttactcaagtttcagtggcttcattgttacaagaaaggggggaagtgagaaactttaataggctgtgatttagaaccactgctgattaacctttggccagtatgggtcagggaaggtgaacatgaaacactgcacagtaggttgtatcaatgctataaaac